European Patent Application EP 4 269 587 A2, published November 1, 2023. Title: Modulation of microRNAs against myotonic dystrophy Type 1 and microRNA antagonists therefor. Applicant: UNIVERSITAT DE VALENCIA. The sequence listing filed with the application follows.

SEQUENCE LISTING (104 sequences)

SEQ ID NO: 1 - RNA, 21 nt, synthetic construct
  misc_feature 1..21: note = Complementary sequence to the human miR-218-5p, base for the generation of inhibitors thereof
  source 1..21: mol_type = other RNA
acatggttagatcaagcacaa

SEQ ID NO: 2 - RNA, 21 nt, synthetic construct
  misc_feature 1..21: note = Complementary sequence to miR-23b-3p, base for the generation of Inhibitors thereof
  source 1..21: mol_type = other RNA
ggtaatccctggcaatgtgat

SEQ ID NO: 3 - RNA, 21 nt, Homo sapiens
  misc_feature 1..21: note = /note="Mature human microRNA miR-218-5p"
  misc_feature 2..8: note = /note="Seed Region"
  source 1..21: mol_type = other RNA
ttgtgcttgatctaaccatgt

SEQ ID NO: 4 - RNA, 21 nt, Homo sapiens
  misc_feature 1..21: note = /note="Mature human microRNA miR-23b-3p"
  misc_feature 2..8: note = /note="Seed Region"
  source 1..21: mol_type = other RNA
atcacattgccagggattacc

SEQ ID NO: 5 - DNA, 699 bp, synthetic construct
  misc_feature 1..699: note = Plasmid Insert (product No. SC400649) that encodes the RNA hsa-miR7 (MI0000265) with hairpin loop that originates hsa-miR-7-5p
  misc_feature 293..402: note = /note="Sequence corresponding to the RNA hsa-miR-7 (MI0000265) with hairpin loop that originates the hsa-miR-7-5p"
  misc_feature 324..346: note = /note="Part corresponding to mature hsa-miR-7-5p (MIMAT0000252)"
  source 1..699: mol_type = other DNA
ctggagtgagctgtgattgcaccactgcactacagcctgggtgacagagcaagaccctgtctcaccaaaacaaaacaaaacaactgtgtccattatagaaagtagaacactccagaaaaaagggaaaagtaagaaaaaataatttctccagggaattctgaggtgaggagaggtgttcaaagatgaacttagtaataggagcggagacaacgcctcgcctgaaggagcatccagaccgctgacctggtggcgaggggaggggggtggtcctcgaacgccttgcagaactggcctggatacagagtggaccggctggccccatctggaagactagtgattttgttgttgtcttactgcgctcaacaacaaatcccagtctacctaatggtgccagccatcgcagcggggtgcaggaaatgggggcagcccccctttttggctatccttccacgtgttcttttttgtatcttttgtgtttcctagaaaacatctcaggtcaccaccctaaacacccatcggcagactcttccagaaacatggacaaactatggtgtgagcagggaagtggggcagggtctctgttttcagggagcagtggactgcttccataccactacctgaagggcagggggagaaaaaccctccttaattactaattcccccaacaatcactttggggcacctataatggaggcacct

SEQ ID NO: 6 - DNA, 650 bp, synthetic construct
  misc_feature 1..650: note = Plasmid Insert (product No. SC400295) that encodes the RNA hsa-miR-23b (MI0000439) with hairpin loop that originates the mature hsa-miR-23b-3p
  misc_feature 281..377: note = /note="Part corresponding to the RNA hsa-miR-23b (MI0000439) with hairpin loop that originates the mature hsa-miR-23b-3p"
  misc_feature 299..320: note = /note="Part corresponding to the mature hsa-miR-23b-3p (MIMAT0000418)"
  source 1..650: mol_type = other DNA
gaggcagtaaactaatagcaaggacagctgcctttagcaattgtgtgtgtcgcatggccggtccctgcatttttcttcagttccaaagctgcactggcatttttatggtcatctctggagtccctttgattcaagaaattatacctctaggatgccaactaaacgaacaacaaacagaaactccacctgtttgctagcataacaggcgtgaaggcggcagtgtcgccggcgtccttccgcggaagcccagtgtgtgcagacagcacggggtggcgctgctctcaggtgctctggctgcttgggttcctggcatgctgatttgtgacttaagattaaaatcacattgccagggattaccacgcaaccacgaccttggctgctcctccagaaaccgtggtcgcgctcactgcagattggagaacaggtgcatctcgtagctcttctttggaaacaaaagaagccaccagctgaggaagatgctcaccggtcaccgtccctttatttatgcccagcgatgacctctctaacaaggtgcagagcttagctgattggtgaacagtgattggtttccgctttgttcacagtggctaagttctgcacctgaagagaaggtgagatggggacagttaagttggagccgctggggcaga

SEQ ID NO: 7 - DNA, 665 bp, synthetic construct
  misc_feature 1..665: note = Plasmid Insert (product No. SC400179) that encodes the RNA hsa-miR-146b (MI0003129) with hairpin loop that originates hsa-miR-146b
  misc_feature 294..366: note = /note="Part corresponding to the RNA hsa-miR-146b (MI0003129) with loop hairpin loop that originates the hsa-miR-146b"
  misc_feature 302..323: note = /note="Part corresponding to the mature hsa-miR-146b (MIMAT0002809)"
  source 1..665: mol_type = other DNA
aacacatctgggcaggaagcgacagatggatccctgccatggccctgagccccctcccctcttaacctactccaattcctgttggaatttatggaactcctgtccatttccttagctgtgggcccccattttcagctccaagctcagaccctccctggaataggagttctcttggtatcacaagttccttatgtgacccatcctgggcctcaacttactcatcctgggaacgggagacgattcacagaagaaagcatgcaagagcagcgtccaggctgaaagaactttggccacctggcactgagaactgaattccataggctgtgagctctagcaatgccctgtggactcagttctggtgcccggcagtgctacaacatcaatgccaaggccgtggggcagctgatggtttgggctcccaacttcccagccaggtgcttctgcaggcccacatcttgcccactggccaaacctttaaataactttgactcgggctactcttatgctcaaagacgtcaggggctctcccaaatctctttaccctgccagaaagtcttctatagtacggcctccacttagctttcacgcctgatcttccatcgcatcctgctcataacctgccactagtgaacccctgctgctccggctccacacttctcatgctg

SEQ ID NO: 8 - DNA, 702 bp, synthetic construct
  misc_feature 1..702: note = Plasmid Insert (product No. SC400283) that encodes the RNA hsa-miR-218 (MI0000295) with hairpin loop that originates hsa-miR-218-5p
  misc_feature 299..408: note = /note="Part corresponding to the RNA hsa-miR-218 (MI0000295) with hairpin loop that originates the hsa-miR-218-5p"
  misc_feature 324..343: note = /note="Part corresponding to the mature hsa-miR-218-5p (MIMAT0000275)"
  source 1..702: mol_type = other DNA
gtgataggatcacagatgtctgagtgttctttctttccttgggaaggaaccatgctgtcctgaagctcccgagtatgggcatccagtgatttccctcccgttcttctcccttcctactgtgtctccctggggtggggcacaagggcagcagggctgcaatcttcggaagtgttccagtggaaccccactcctgatactaatcacgctcagtgggggcctgctccggcttccgcttctccacgctgcttcctctgagcgctcctgtcctctctctgacgctgcttcctgaccttgactctgaccagtcgctgcggggctttcctttgtgcttgatctaaccatgtggtggaacgatggaaacggaacatggttctgtcaagcaccgcggaaagcaccgtgctctcctgcagcatggcccgccaccgccgccaccaccgctggacacctctcctctgctctggagcaccgcagcccaccacctgccagacccacctctcccagtctcaactcaccaaaggcaggagggtaggagtctcaaaggatgcagatacagagggaaatgggtctggagaagcaccctggggaaagagatctgtatccacatctctttcccaaaatggagtcaccctcccccaaatctagtctggatgtcagacaaggagtaataactaggttcaagctcagaaactactgtgtctcttc

SEQ ID NO: 9 - DNA, 625 bp, synthetic construct
  misc_feature 1..625: note = Plasmid Insert (product No. SC400368) that encodes the RNA hsa-miR-372 (MI0000780) with hairpin loop that originates hsa-miR-372
  misc_feature 278..344: note = /note="Part corresponding to the RNA hsa-miR-372(MI0000780) with hairpin loop that originates the hsa-miR-372-3p"
  misc_feature 319..341: note = /note="Part corresponding to the mature hsa-miR-372-3p (MIMAT0000724)"
  source 1..625: mol_type = other DNA
gcctcttctgatgggtaagtgcttccacttgcgatcgccgccttgccgcatcccctcagcctgtggcactcaaactgtgggggcactttctgctctctggtgaaagtgccgccatcttttgagtgttaccgcttgagaagactcaacctgcggagaagataccattttgattgggtgagggggcgggtagcaggatggccctagaccctgcctatggccgtttcctcgtgatataaatttcttggccggggctcttgcagatggagctgctcaccctgtgggcctcaaatgtggagcactattctgatgtccaagtggaaagtgctgcgacatttgagcgtcaccggtgacgcccatatcaacggatgccgtggagctcggtcttctgcaggaactaaagagcctgtggtttcgattcccagccggaaactgtcttgggtacaggtcccttacagcgtctggctgtaatggctccggaaaacctggggaagggaagggggcctcctgggctctcacctgacacaactaagggaatctgggttagatggtgaaaggaagagaaggttcagagggcggctgtgcgcctgcgccgggcgcggcggctcacacctgtaatcccagcacg

SEQ ID NO: 10 - RNA, 21 nt, synthetic construct
  misc_feature 1..21: note = Base sequence of the antagomiR-218-5p, which includes modified nucleotides -
  modified_base 1..2: mod_base = OTHER; note = /mod_base="OTHER" /note="Nucleotide bound to the next by phosphorothioate group"
  modified_base 3..4: mod_base = OTHER; note = /mod_base="OTHER" /note="Nucleotide bound to the next by phosphorothioate group"
  modified_base 1..21: mod_base = OTHER; note = /mod_base="OTHER" /note="Nucleotide with 2'-O-methyl (2'-methoxy) modification"
  modified_base 18..20: mod_base = OTHER; note = /mod_base="OTHER" /note="Nucleotide bound to the next by a phosphorothioate bond"
  modified_base 21: mod_base = OTHER; note = /mod_base="OTHER" /note="Nucleotide bound to 4 cholesterol groups; the nucleotide bond to the first cholesterol group is through a phosphorothioate group"
  source 1..21: mol_type = other RNA
acatggttagatcaagcacaa

SEQ ID NO: 11 - RNA, 21 nt, synthetic construct
  misc_feature 1..21: note = antagomir23b-5p sequence
  modified_base 1..2: mod_base = OTHER; note = /mod_base="OTHER" /note="Nucleotide bound to the next by phosphorothioate group"
  modified_base 2..3: mod_base = OTHER; note = /mod_base="OTHER" /note="Nucleotide bound to the next by phosphorothioate group"
  modified_base 1..21: mod_base = OTHER; note = /mod_base="OTHER" /note="Nucleotide with 2'-O-methyl (2'-methoxy) modification"
  modified_base 18..20: mod_base = OTHER; note = /mod_base="OTHER" /note="Nucleotide bound to the next by a phosphorothioate bond"
  modified_base 21: mod_base = OTHER; note = /mod_base="OTHER" /note="Nucleotide bound to 4 cholesterol groups; the nucleotide bond to the first cholesterol group is through a phosphorothioate group"
  source 1..21: mol_type = other RNA
ggtaatccctggcaatgtgat

SEQ ID NO: 12 - RNA, 21 nt, Homo sapiens
  misc_feature 1..21: note = /note="mature microRNA-23b: hsa-miR-23b-3p (MIMAT0000418)"
  source 1..21: mol_type = other RNA
atcacattgccagggattacc

SEQ ID NO: 13 - RNA, 21 nt, Homo sapiens
  misc_feature 1..21: note = /note="mature hsa-miR-218-5p (MIMAT0000275)"
  source 1..21: mol_type = other RNA
ttgtgcttgatctaaccatgt

SEQ ID NO: 14 - DNA, 20 bp, synthetic construct
  misc_feature 1..20: note = Direct primer of gene PCR transcript amplification GAPDH
  source 1..20: mol_type = other DNA
catcttccaggagcgagatc

SEQ ID NO: 15 - DNA, 21 bp, synthetic construct
  misc_feature 1..21: note = Inverse primer of gene PCR transcript amplification GAPDH
  source 1..21: mol_type = other DNA
gttcacacccatgacgaacat

SEQ ID NO: 16 - DNA, 24 bp, synthetic construct
  misc_feature 1..24: note = Direct primer of gene PCR transcript amplification cTNT
  source 1..24: mol_type = other DNA
atagaagaggtggtggaagagtac

SEQ ID NO: 17 - DNA, 24 bp, synthetic construct
  misc_feature 1..24: note = Inverse primer of gene PCR transcript amplification cTNT
  source 1..24: mol_type = other DNA
gtctcagcctctgcttcagcatcc

SEQ ID NO: 18 - DNA, 20 bp, synthetic construct
  misc_feature 1..20: note = Direct primer of IR gene PCR transcript amplification
  source 1..20: mol_type = other DNA
tgctgctcctgtccaaagac

SEQ ID NO: 19 - DNA, 19 bp, synthetic construct
  misc_feature 1..19: note = Inverse primer of IR gene PCR transcript amplification
  source 1..19: mol_type = other DNA
gaagtgttggggaaagctg

SEQ ID NO: 20 - DNA, 24 bp, synthetic construct
  misc_feature 1..24: note = Direct primer of gene PCR transcript amplification BIN1
  source 1..24: mol_type = other DNA
ctcaaccagaacctcaatgatgtg

SEQ ID NO: 21 - DNA, 21 bp, synthetic construct
  misc_feature 1..21: note = Inverse primer of gene PCR transcript amplification BIN1
  source 1..21: mol_type = other DNA
ctgagatggggacttggggag

SEQ ID NO: 22 - DNA, 22 bp, synthetic construct
  misc_feature 1..22: note = Direct primer of gene PCR transcript amplification DMD
  source 1..22: mol_type = other DNA
gtgaggaagatcttctcagtcc

SEQ ID NO: 23 - DNA, 21 bp, synthetic construct
  misc_feature 1..21: note = Inverse primer of gene PCR transcript amplification DMD
  source 1..21: mol_type = other DNA
ctccatcgctctgcccaaatc

SEQ ID NO: 24 - DNA, 21 bp, synthetic construct
  misc_feature 1..21: note = Direct primer of gene PCR transcript amplification SERCA1
  source 1..21: mol_type = other DNA
gatgatcttcaagctccgggc

SEQ ID NO: 25 - DNA, 20 bp, synthetic construct
  misc_feature 1..20: note = Inverse primer of gene PCR transcript amplification SERCA1
  source 1..20: mol_type = other DNA
cagctctgcctgaagatgtg

SEQ ID NO: 26 - RNA, 22 nt, Drosophila melanogaster
  misc_feature 1..22: note = /note="Mature microRNA dme-mR-92a-3p (MIMAT0000334)"
  source 1..22: mol_type = other RNA
cattgcacttgtcccggcctat

SEQ ID NO: 27 - RNA, 22 nt, Drosophila melanogaster
  misc_feature 1..22: note = /note="Mature microRNA dme-miR-100-5p (MIMAT0000357)"
  source 1..22: mol_type = other RNA
aacccgtaaatccgaacttgtg

SEQ ID NO: 28 - RNA, 23 nt, Drosophila melanogaster
  misc_feature 1..23: note = /note="Mature microRNA dme-miR-124-3p (MIMAT0000351)"
  source 1..23: mol_type = other RNA
taaggcacgcggtgaatgccaag

SEQ ID NO: 29 - RNA, 23 nt, Drosophila melanogaster
  misc_feature 1..23: note = /note="Mature microRNA dme-miR-277-3p (MIMAT0000338)"
  source 1..23: mol_type = other RNA
taaatgcactatctggtacgaca

SEQ ID NO: 30 - RNA, 23 nt, Drosophila melanogaster
  misc_feature 1..23: note = /note="Mature microRNA dme-miR-304-5p (MIMAT0000390)"
  source 1..23: mol_type = other RNA
taatctcaatttgtaaatgtgag

SEQ ID NO: 31 - DNA, 25 bp, synthetic construct
  misc_feature 1..25: note = Direct primer of qRT-PCR of mbl
  source 1..25: mol_type = other DNA
ttgaatcaaaattatagcccaagct

SEQ ID NO: 32 - DNA, 21 bp, synthetic construct
  misc_feature 1..21: note = Inverse primer of qRT-PCR of mbl
  source 1..21: mol_type = other DNA
cgattttgctcgttagcgttt

SEQ ID NO: 33 - DNA, 27 bp, synthetic construct
  misc_feature 1..27: note = Direct primer of qRT-PCR of mblA
  source 1..27: mol_type = other DNA
cagacaccgaaatactctctacaaaca

SEQ ID NO: 34 - DNA, 30 bp, synthetic construct
  misc_feature 1..30: note = Inverse primer of qRT-PCR of mbl
  source 1..30: mol_type = other DNA
aaaatcaggagtaaacaaatacacgtagac

SEQ ID NO: 35 - DNA, 26 bp, synthetic construct
  misc_feature 1..26: note = Direct primer of qRT-PCR of mblB
  source 1..26: mol_type = other DNA
cacacatccagatatgctacttacca

SEQ ID NO: 36 - DNA, 22 bp, synthetic construct
  misc_feature 1..22: note = Inverse primer of qRT-PCR of mblB
  source 1..22: mol_type = other DNA
tgagcgatttcgattgattttg

SEQ ID NO: 37 - DNA, 23 bp, synthetic construct
  misc_feature 1..23: note = Direct primer of qRT-PCR of mblC
  source 1..23: mol_type = other DNA
cagcaaacacacatcacctacca

SEQ ID NO: 38 - DNA, 23 bp, synthetic construct
  misc_feature 1..23: note = Inverse primer of qRT-PCR of mblC
  source 1..23: mol_type = other DNA
ctatcgagcaggaggatgaagag

SEQ ID NO: 39 - DNA, 20 bp, synthetic construct
  misc_feature 1..20: note = Direct primer of qRT-PCR of mblD
  source 1..20: mol_type = other DNA
gcctctggaaaatgctgcaa

SEQ ID NO: 40 - DNA, 20 bp, synthetic construct
  misc_feature 1..20: note = Inverse primer of qRT-PCR of mblD
  source 1..20: mol_type = other DNA
cagcaaccgcaaaagagctt

SEQ ID NO: 41 - DNA, 19 bp, synthetic construct
  misc_feature 1..19: note = Direct primer of qRT-PCR of Serca
  source 1..19: mol_type = other DNA
gcagatgttcctgatgtcg

SEQ ID NO: 42 - DNA, 19 bp, synthetic construct
  misc_feature 1..19: note = Inverse primer of qRT-PCR of Serca
  source 1..19: mol_type = other DNA
cgtcctccttcacattcac

SEQ ID NO: 43 - DNA, 20 bp, synthetic construct
  misc_feature 1..20: note = Direct primer of qRT-PCR of Cyp6w1
  source 1..20: mol_type = other DNA
ttgcgcacaaaaatctctcc

SEQ ID NO: 44 - DNA, 20 bp, synthetic construct
  misc_feature 1..20: note = Inverse primer of qRT-PCR of Cyp6w1
  source 1..20: mol_type = other DNA
gtcctgcaagttctttccaa

SEQ ID NO: 45 - DNA, 26 bp, synthetic construct
  misc_feature 1..26: note = Direct primer of qRT-PCR of Rp49
  source 1..26: mol_type = other DNA
ggatcgatatgctaagctgtcgcaca

SEQ ID NO: 46 - DNA, 24 bp, synthetic construct
  misc_feature 1..24: note = Inverse primer of qRT-PCR of Rp49
  source 1..24: mol_type = other DNA
ggtgcgcttgttcgatccgtaacc

SEQ ID NO: 47 - DNA, 20 bp, synthetic construct
  misc_feature 1..20: note = Direct primer of qRT-PCR of Fhos
  source 1..20: mol_type = other DNA
gtcatggagtcgagcagtga

SEQ ID NO: 48 - DNA, 20 bp, synthetic construct
  misc_feature 1..20: note = Inverse primer of qRT-PCR of Phos
  source 1..20: mol_type = other DNA
tgtgatgcgggtatctacga

SEQ ID NO: 49 - DNA, 18 bp, synthetic construct
  misc_feature 1..18: note = Direct primer of qRT-PCR of Tnt
  source 1..18: mol_type = other DNA
cgacgatgaagagtacac

SEQ ID NO: 50 - DNA, 22 bp, synthetic construct
  misc_feature 1..22: note = Inverse primer of qRT-PCR of Tnt
  source 1..22: mol_type = other DNA
actcggtgatgtattctttcag

SEQ ID NO: 51 - DNA, 3438 bp, Homo sapiens
  3'UTR 1..3438: note = /note="3'UTR region of the transcript of the MBNL1 gene (NM_ 207297.1) inserted in the plasmid pEZX-MT05"
  misc_feature 3130..3150: note = /note="MiR-23b binding region"
  source 1..3438: mol_type = other DNA
ccacaagtatgttacccagatgtagaattttcatcactaaacaatcatgctaaagaggaaaggacagtgtgcttggttagagtaaaggacgaggtcattagccatattgtatatatcgtcaagcaacacacacaaaagttcctcagccacaagacatccacatattgcatgttaaccagaagaaaagacaacattttccggaaatccactgcacactgttgcctatacactttgtacatttaattgatatttgtgctgaggtgatattcctgtctaaaagaacaacattgtctttcttttctagcacagagttatgcattcaaagatgcatacctagttagtttcctatatattcatgccatcttgaaaagacagactatggtgtaaccatgattctattatgtattggtacgtctgtagaccaagatataattttttaaaaataagtttatttctttcaaggtttacaaataacaaaggtgcaccttgtatttaaaattgccattatagatgagagcgtgcatgcacagtcatttttgtttaagagtaatatttttaatgtaatagattgtaagacgtggtgagggagggatctgacagagatgaatgtgccaagcaaaaccacaactgtgtatattttaaagcacatcatggctttaagtaccatgttgttaaggattctcatgaagtgccatagactgtacatcaaattagagtattatttcttcagtgttattgttttcagagccacattttgttgcatatttgctagtactaatcagtcaaagggcaccattctttttttttttttttgaaaccaaagctgtctcagaaatggccaatttaactttacagtaacaatagacagcacaacacaaactctctcaatacagataaactcacacatactggagatatatatataatagatatatataaaattattttaatgcattgtagtgtaatatttatgcatactatactgtataacatgttattcaaaagggattgccatttctgagacacagtaacaaaaaaatgaggaaattattttgcttctatttatagcctctgtcaaaagtcaaaagactataaatgctttgcaaaaatggtttcacgtttgcttaaatgcttcatcacagtcacattcaaaatagtgactctaaacaaagaagaaagcagcactgtcatcagatgcatgataaaccaaaatatgaaaatgggaaatgtttaattaacctagtaattgggtgggttaagtacatgggtgaattttatatgtgatttttgttttgttttgttttgttcagattaactgcttatagccttagaaagccttttacaaaattaaaaaaaaaatagatgtgcattcagtttttaagaatggaatcatccaaaggaattcctttttttgaggtttggatgttgcagctagtaaaggatatttttgctctgttcagcagttctaaaaattgctgaagtaggggccaggtcactggtagttatagtatggaatgggagaagtgaaagttcagttatagaactttccatacttccaagtttactgcaagtttttatgcttgagagagatgctttctaatataagactgatgtgttgattttactgattgtactgtacatctattaaagccttagattattacattacgggttggaacccataccaatgtaatttcaatcgtgttaagaaagtaatggtgacttcacatgttattgtagttagttacattatagaatattacttatttttcttgttaaaatgtagtttttcatttcctacatttattagattttcattttctattaacaattgaataccatttcagtttatagacttgttttattagattttaccaatgaatttttcaaaatacaaaaaaaagtagtttttccttcataacatactcagttttgaattacatgtagtgtcacatgaatattcgtattgttaactaaatgatttatattttactgatttaatattacagtgtaagaatgtcagtcattgttagttcttgtctagttttcattaaaagaacaaagatcttttatatggatatcttataaatatataatcattgctaagtaagaagttaagttgttgctatcgcaacaatcctggcagacaattgagtaatattttgatgatttattttgtttgtaattagttattataagaagatctagatcctagatattagaataaaatttattttctactgtatccatttcaaatgttaaaatattgtttaatatttttgaaatccctgagtatcaggccttgttataaataagctgcataatcaataaatagaacaagggactttttgttgataatccaaatactcaaagtttacgtaatgaaaattatagcgtgtgtgcaaactcttgagggttgattatgctgcaatttagcatgttggaacgtctagggagaaggttgactttttgcacttctgtatatagtcaaaagagagaaacctgtataatagtaagatcttattttgaataaaaacgtctataattacaaggagttttgttaaggctaatacaatgacagactgagcaaaattgcttgcaaaagtggcacagagttagcactccataccccttcaaacatgttgctttgctttcttgtggacagcttgtagtttgccaggattttttcagctggaaagatacgccatcctttcaaaccctcatgactgacaaaaactccatggggccaaatctgcctgaagatcattaccaaaaatagcaggtacttctaccattaaggtgaaatcatggatcagatattccttacatttttcaaaactactgcatgtttaaaacttcaacaaaaaaagagagaaagaactatactaagaacatatattattcagatcagtttctgccaatttcagtggtttattgttcacaaaaaaatcttcaaaacaagtattgactttcacaaaatttaaatcataaacaggcaaaccaaacagcacactgtagctatagttgttatgtgattgttttttaattgctgtaggatcctgttctttcagcaggtgaaaaataaaacgcagttcaaatttcatggttttaattttcaactcagaagcactcaaaaatgcaaaatgtgataatgggcacttgtttaaaagaattagtgtatccagccttcactccagctggttaaaaatgttgcacttatcagcaaccctaccactttcatctgctgaaaggacaaatgtgcttggttttactattatgtaatcacaacttactttctgcttgtagttgcttaaaattatgtattttgtcttgggctgcaatttgttttatgcttattttattattactgcagtagttgactttgctgtatggaaaaataaagtgaaattgccctaataaaacttctctttcttaagt

SEQ ID NO: 52 - DNA, 3430 bp, synthetic construct
  misc_feature 1..3430: note = 3'UTR region of MBNL1 with seed region of miR-23b deleted (3'UTR MUT-23b)
  misc_feature 3142..3143: note = /note="Nucleotides flanking the fragment of the deleted seed region ."
  source 1..3430: mol_type = other DNA
ccacaagtatgttacccagatgtagaattttcatcactaaacaatcatgctaaagaggaaaggacagtgtgcttggttagagtaaaggacgaggtcattagccatattgtatatatcgtcaagcaacacacacaaaagttcctcagccacaagacatccacatattgcatgttaaccagaagaaaagacaacattttccggaaatccactgcacactgttgcctatacactttgtacatttaattgatatttgtgctgaggtgatattcctgtctaaaagaacaacattgtctttcttttctagcacagagttatgcattcaaagatgcatacctagttagtttcctatatattcatgccatcttgaaaagacagactatggtgtaaccatgattctattatgtattggtacgtctgtagaccaagatataattttttaaaaataagtttatttctttcaaggtttacaaataacaaaggtgcaccttgtatttaaaattgccattatagatgagagcgtgcatgcacagtcatttttgtttaagagtaatatttttaatgtaatagattgtaagacgtggtgagggagggatctgacagagatgaatgtgccaagcaaaaccacaactgtgtatattttaaagcacatcatggctttaagtaccatgttgttaaggattctcatgaagtgccatagactgtacatcaaattagagtattatttcttcagtgttattgttttcagagccacattttgttgcatatttgctagtactaatcagtcaaagggcaccattctttttttttttttttgaaaccaaagctgtctcagaaatggccaatttaactttacagtaacaatagacagcacaacacaaactctctcaatacagataaactcacacatactggagatatatatataatagatatatataaaattattttaatgcattgtagtgtaatatttatgcatactatactgtataacatgttattcaaaagggattgccatttctgagacacagtaacaaaaaaatgaggaaattattttgcttctatttatagcctctgtcaaaagtcaaaagactataaatgctttgcaaaaatggtttcacgtttgcttaaatgcttcatcacagtcacattcaaaatagtgactctaaacaaagaagaaagcagcactgtcatcagatgcatgataaaccaaaatatgaaaatgggaaatgtttaattaacctagtaattgggtgggttaagtacatgggtgaattttatatgtgatttttgttttgttttgttttgttcagattaactgcttatagccttagaaagccttttacaaaattaaaaaaaaaatagatgtgcattcagtttttaagaatggaatcatccaaaggaattcctttttttgaggtttggatgttgcagctagtaaaggatatttttgctctgttcagcagttctaaaaattgctgaagtaggggccaggtcactggtagttatagtatggaatgggagaagtgaaagttcagttatagaactttccatacttccaagtttactgcaagtttttatgcttgagagagatgctttctaatataagactgatgtgttgattttactgattgtactgtacatctattaaagccttagattattacattacgggttggaacccataccaatgtaatttcaatcgtgttaagaaagtaatggtgacttcacatgttattgtagttagttacattatagaatattacttatttttcttgttaaaatgtagtttttcatttcctacatttattagattttcattttctattaacaattgaataccatttcagtttatagacttgttttattagattttaccaatgaatttttcaaaatacaaaaaaaagtagtttttccttcataacatactcagttttgaattacatgtagtgtcacatgaatattcgtattgttaactaaatgatttatattttactgatttaatattacagtgtaagaatgtcagtcattgttagttcttgtctagttttcattaaaagaacaaagatcttttatatggatatcttataaatatataatcattgctaagtaagaagttaagttgttgctatcgcaacaatcctggcagacaattgagtaatattttgatgatttattttgtttgtaattagttattataagaagatctagatcctagatattagaataaaatttattttctactgtatccatttcaaatgttaaaatattgtttaatatttttgaaatccctgagtatcaggccttgttataaataagctgcataatcaataaatagaacaagggactttttgttgataatccaaatactcaaagtttacgtaatgaaaattatagcgtgtgtgcaaactcttgagggttgattatgctgcaatttagcatgttggaacgtctagggagaaggttgactttttgcacttctgtatatagtcaaaagagagaaacctgtataatagtaagatcttattttgaataaaaacgtctataattacaaggagttttgttaaggctaatacaatgacagactgagcaaaattgcttgcaaaagtggcacagagttagcactccataccccttcaaacatgttgctttgctttcttgtggacagcttgtagtttgccaggattttttcagctggaaagatacgccatcctttcaaaccctcatgactgacaaaaactccatggggccaaatctgcctgaagatcattaccaaaaatagcaggtacttctaccattaaggtgaaatcatggatcagatattccttacatttttcaaaactactgcatgtttaaaacttcaacaaaaaaagagagaaagaactatactaagaacatatattattcagatcagtttctgccaatttcagtggtttattgttcacaaaaaaatcttcaaaacaagtattgactttcacaaaatttaaatcataaacaggcaaaccaaacagcacactgtagctatagttgttatgtgattgttttttaattgctgtaggatcctgttctttcagcaggtgaaaaataaaacgcagttcaaatttcatggttttaattttcaactcagaagcactcaaaaatgcaaaatgggcacttgtttaaaagaattagtgtatccagccttcactccagctggttaaaaatgttgcacttatcagcaaccctaccactttcatctgctgaaaggacaaatgtgcttggttttactattatgtaatcacaacttactttctgcttgtagttgcttaaaattatgtattttgtcttgggctgcaatttgttttatgcttattttattattactgcagtagttgactttgctgtatggaaaaataaagtgaaattgccctaataaaacttctctttcttaagt

SEQ ID NO: 53 - DNA, 3438 bp, synthetic construct
  misc_feature 1..3438: note = Insert of plasmid pEZX-MT05 with the 3'UTR of MBNL 1 modified (3 UTR PM-23b)
  misc_feature 3130..3150: note = /note="Region modified for perfect complementarity with miR-23b"
  source 1..3438: mol_type = other DNA
ccacaagtatgttacccagatgtagaattttcatcactaaacaatcatgctaaagaggaaaggacagtgtgcttggttagagtaaaggacgaggtcattagccatattgtatatatcgtcaagcaacacacacaaaagttcctcagccacaagacatccacatattgcatgttaaccagaagaaaagacaacattttccggaaatccactgcacactgttgcctatacactttgtacatttaattgatatttgtgctgaggtgatattcctgtctaaaagaacaacattgtctttcttttctagcacagagttatgcattcaaagatgcatacctagttagtttcctatatattcatgccatcttgaaaagacagactatggtgtaaccatgattctattatgtattggtacgtctgtagaccaagatataattttttaaaaataagtttatttctttcaaggtttacaaataacaaaggtgcaccttgtatttaaaattgccattatagatgagagcgtgcatgcacagtcatttttgtttaagagtaatatttttaatgtaatagattgtaagacgtggtgagggagggatctgacagagatgaatgtgccaagcaaaaccacaactgtgtatattttaaagcacatcatggctttaagtaccatgttgttaaggattctcatgaagtgccatagactgtacatcaaattagagtattatttcttcagtgttattgttttcagagccacattttgttgcatatttgctagtactaatcagtcaaagggcaccattctttttttttttttttgaaaccaaagctgtctcagaaatggccaatttaactttacagtaacaatagacagcacaacacaaactctctcaatacagataaactcacacatactggagatatatatataatagatatatataaaattattttaatgcattgtagtgtaatatttatgcatactatactgtataacatgttattcaaaagggattgccatttctgagacacagtaacaaaaaaatgaggaaattattttgcttctatttatagcctctgtcaaaagtcaaaagactataaatgctttgcaaaaatggtttcacgtttgcttaaatgcttcatcacagtcacattcaaaatagtgactctaaacaaagaagaaagcagcactgtcatcagatgcatgataaaccaaaatatgaaaatgggaaatgtttaattaacctagtaattgggtgggttaagtacatgggtgaattttatatgtgatttttgttttgttttgttttgttcagattaactgcttatagccttagaaagccttttacaaaattaaaaaaaaaatagatgtgcattcagtttttaagaatggaatcatccaaaggaattcctttttttgaggtttggatgttgcagctagtaaaggatatttttgctctgttcagcagttctaaaaattgctgaagtaggggccaggtcactggtagttatagtatggaatgggagaagtgaaagttcagttatagaactttccatacttccaagtttactgcaagtttttatgcttgagagagatgctttctaatataagactgatgtgttgattttactgattgtactgtacatctattaaagccttagattattacattacgggttggaacccataccaatgtaatttcaatcgtgttaagaaagtaatggtgacttcacatgttattgtagttagttacattatagaatattacttatttttcttgttaaaatgtagtttttcatttcctacatttattagattttcattttctattaacaattgaataccatttcagtttatagacttgttttattagattttaccaatgaatttttcaaaatacaaaaaaaagtagtttttccttcataacatactcagttttgaattacatgtagtgtcacatgaatattcgtattgttaactaaatgatttatattttactgatttaatattacagtgtaagaatgtcagtcattgttagttcttgtctagttttcattaaaagaacaaagatcttttatatggatatcttataaatatataatcattgctaagtaagaagttaagttgttgctatcgcaacaatcctggcagacaattgagtaatattttgatgatttattttgtttgtaattagttattataagaagatctagatcctagatattagaataaaatttattttctactgtatccatttcaaatgttaaaatattgtttaatatttttgaaatccctgagtatcaggccttgttataaataagctgcataatcaataaatagaacaagggactttttgttgataatccaaatactcaaagtttacgtaatgaaaattatagcgtgtgtgcaaactcttgagggttgattatgctgcaatttagcatgttggaacgtctagggagaaggttgactttttgcacttctgtatatagtcaaaagagagaaacctgtataatagtaagatcttattttgaataaaaacgtctataattacaaggagttttgttaaggctaatacaatgacagactgagcaaaattgcttgcaaaagtggcacagagttagcactccataccccttcaaacatgttgctttgctttcttgtggacagcttgtagtttgccaggattttttcagctggaaagatacgccatcctttcaaaccctcatgactgacaaaaactccatggggccaaatctgcctgaagatcattaccaaaaatagcaggtacttctaccattaaggtgaaatcatggatcagatattccttacatttttcaaaactactgcatgtttaaaacttcaacaaaaaaagagagaaagaactatactaagaacatatattattcagatcagtttctgccaatttcagtggtttattgttcacaaaaaaatcttcaaaacaagtattgactttcacaaaatttaaatcataaacaggcaaaccaaacagcacactgtagctatagttgttatgtgattgttttttaattgctgtaggatcctgttctttcagcaggtgaaaaataaaacgcagttcaaatttcatggttttaattttcaactcagaagcaggtaatccctggcaatgtgataatgggcacttgtttaaaagaattagtgtatccagccttcactccagctggttaaaaatgttgcacttatcagcaaccctaccactttcatctgctgaaaggacaaatgtgcttggttttactattatgtaatcacaacttactttctgcttgtagttgcttaaaattatgtattttgtcttgggctgcaatttgttttatgcttattttattattactgcagtagttgactttgctgtatggaaaaataaagtgaaattgccctaataaaacttctctttcttaagt

SEQ ID NO: 54 - DNA, 2783 bp, Homo sapiens
  3'UTR 1..2783: note = /note="3'UTR of the gene MBNL2 (NM_ 44778.2) inserted in the plasmid pEZX-MT05"
  misc_feature 582..601: note = /note="miR-218 binding region 1"
  misc_feature 646..665: note = /note="MiR-23b binding region"
  misc_feature 1368..1388: note = /note="miR-218 binding region 2"
  misc_feature 2085..2105: note = /note="miR-218 binding region 1"
  source 1..2783: mol_type = other DNA
tcagcagaaacggaatggaatgccaagaatctgcattgagaataactaaacattgttactgtacatactatcctgtttcctcctcaatagaattgccacaaactgcatgctaaataaagatgtagttcttctggacagaccacaactctaagaagctagtgctgctatctcatatatgagtattaaatatggtatgcttagtatattccaacctaagatagttaactacctgagaccagctgtgatgtttaaagacataaaggataaagtttacttttaaagggtttctaaacatagtttctgtcctaggaatattgtcttatctccataactatagctgatgcagaaagtccagccagtttactcatttcgattcagaatatttcaaatttagcaataaacaattagcattagttaaaaaagaaacatattccaagggcaggttcgattctagctctaattactgtcatgtcatttacccactggatcaaagggtatgtttcacttcttgacaatataaatgctgcagcaaagatgagaggtgaagtaaaaccgatacctgtcctgcaggtctaaaatttgaatggaaattcaagcacaagtactggggacacatcaaagtgtggtgtttggtttgcctggagatgccacgttgaatcatgtgattctagattaacattaaatagattgaaaaagaaactttgcacggtatgagcttcataccccaccaaacaaagtcttgaaggtattattttacaagtatatttttaaagttgttttataagagagactttgtagaagtgcctagattttgccagacttcatccagcttgacaagattgagaggcccatgccaacagtctaatctaagagattagtctttcaaactcaccatccagttgcctgttacagaataactcttcttaactaaaaacctagtcaaacaaggaagctgtaggtgaggagatctgtataatattctaatttaagtaagtttgagtttagtcactgcaaatttgactgtgactttaatctaaattactatgtaaacaaaaagtagatagtttcactttttaaaaaatccattactgttttgcatttcaaaagttggattaaagggttgtaactgactacagcatggaaaaaaatagttcttttaattctttcaccttaaagcatattttatgtctcaaaagtataaaaaactttaatacaagtacatacatattatatatacacatacatatatatactatatatggatgaaacatattttaatgttgtttacttttttaaatacttggttgatcttcaaggtaatagcgatacaattaaattttgttcagaaagtttgttttaaagtttattttaagcactatcgtaccaaatatttcatatttcacattttatatgttgcacatagcctatacagtacctacatagtttttaaattattgtttaaaaaacaaaacagctgttataaatgaatattatgtgtaattgtttcaaacatccattttctttgtgaacatattagtgattgaagtattttgacttttgagattgaatgtaaaatattttaaatttgggatcatcgcctgttctgaaaactagatgcaccaaccgtatcattatttgtttgaggaaaaaaagaaatctgcattttaattcatgttggtcaaagtcgaattactatctatttatcttatatcgtagatctgataaccctatctaaaagaaagtcacacgctaaatgtattcttacatagtgcttgtatcgttgcatttgttttaatttgtggaaaagtattgtatctaacttgtattactttggtagtttcatctttatgtattattgatatttgtaattttctcaactataacaatgtagttacgctacaacttgcctaaaacattcaaacttgttttcttttttctgtttttttctttgttaattcatttaaactcattgaaaacatagtatacattactaaaaggtaaattatgggaatcactgaaatatttttgtagattaattgttgtaacattgtctttcttttttttcttttgtttcatgattttgatttttaaaattattagcacacaactattttcagccctttaataatggagcatcaaaaacatcacctgtaaccccaagcaaatatagaagactgtattttttactatgatatccattttccagaattgtgattacaatatgcaaagagtcataaatatgccatttacaataaggaggaggcaaggcaaatgcatagatgtacaaatatatgtacaacagattttgctttttatttatttataatgtaattttatagaataattctgggatttgagaggatctaaaactatttttctgtataaatattatttgccaaaagtttgtttatattcagaagtctgactatgatgaataaatcttaaatgctttgtttaattaaaaaacaaaaatcaccaatatccaagacatgaagatatcagttcaacaaatactgtagttaagagactaactctccacttgtatgggaactacatttcactcttggttttcaggatataacagcacttcaccgaaatattctttcagccataccactggtaacatttctactaaatctttctgtaacacttaaagaattccctcattcattaccttacagtgtaaacaggagtctaatttgtatcaatactatgttttggttgtaatattcagttcactcacccaatgtacaaccaatgaaataaaagaagcatttaaaagg

SEQ ID NO: 55 - DNA, 2777 bp, synthetic construct
  misc_feature 1..2777: note = 3'UTR of MBNL2 with seed region of miR-23b deleted (3'UTR MUT-23b)
  misc_feature 659..660: note = /note="Nucleotides flanking the fragment of the deleted seed region of miR-23b"
  source 1..2777: mol_type = other DNA
tcagcagaaacggaatggaatgccaagaatctgcattgagaataactaaacattgttactgtacatactatcctgtttcctcctcaatagaattgccacaaactgcatgctaaataaagatgtagttcttctggacagaccacaactctaagaagctagtgctgctatctcatatatgagtattaaatatggtatgcttagtatattccaacctaagatagttaactacctgagaccagctgtgatgtttaaagacataaaggataaagtttacttttaaagggtttctaaacatagtttctgtcctaggaatattgtcttatctccataactatagctgatgcagaaagtccagccagtttactcatttcgattcagaatatttcaaatttagcaataaacaattagcattagttaaaaaagaaacatattccaagggcaggttcgattctagctctaattactgtcatgtcatttacccactggatcaaagggtatgtttcacttcttgacaatataaatgctgcagcaaagatgagaggtgaagtaaaaccgatacctgtcctgcaggtctaaaatttgaatggaaattcaagcacaagtactggggacacatcaaagtgtggtgtttggtttgcctggagatgccacgttgaatcttctagattaacattaaatagattgaaaaagaaactttgcacggtatgagcttcataccccaccaaacaaagtcttgaaggtattattttacaagtatatttttaaagttgttttataagagagactttgtagaagtgcctagattttgccagacttcatccagcttgacaagattgagaggcccatgccaacagtctaatctaagagattagtctttcaaactcaccatccagttgcctgttacagaataactcttcttaactaaaaacctagtcaaacaaggaagctgtaggtgaggagatctgtataatattctaatttaagtaagtttgagtttagtcactgcaaatttgactgtgactttaatctaaattactatgtaaacaaaaagtagatagtttcactttttaaaaaatccattactgttttgcatttcaaaagttggattaaagggttgtaactgactacagcatggaaaaaaatagttcttttaattctttcaccttaaagcatattttatgtctcaaaagtataaaaaactttaatacaagtacatacatattatatatacacatacatatatatactatatatggatgaaacatattttaatgttgtttacttttttaaatacttggttgatcttcaaggtaatagcgatacaattaaattttgttcagaaagtttgttttaaagtttattttaagcactatcgtaccaaatatttcatatttcacattttatatgttgcacatagcctatacagtacctacatagtttttaaattattgtttaaaaaacaaaacagctgttataaatgaatattatgtgtaattgtttcaaacatccattttctttgtgaacatattagtgattgaagtattttgacttttgagattgaatgtaaaatattttaaatttgggatcatcgcctgttctgaaaactagatgcaccaaccgtatcattatttgtttgaggaaaaaaagaaatctgcattttaattcatgttggtcaaagtcgaattactatctatttatcttatatcgtagatctgataaccctatctaaaagaaagtcacacgctaaatgtattcttacatagtgcttgtatcgttgcatttgttttaatttgtggaaaagtattgtatctaacttgtattactttggtagtttcatctttatgtattattgatatttgtaattttctcaactataacaatgtagttacgctacaacttgcctaaaacattcaaacttgttttcttttttctgtttttttctttgttaattcatttaaactcattgaaaacatagtatacattactaaaaggtaaattatgggaatcactgaaatatttttgtagattaattgttgtaacattgtctttcttttttttcttttgtttcatgattttgatttttaaaattattagcacacaactattttcagccctttaataatggagcatcaaaaacatcacctgtaaccccaagcaaatatagaagactgtattttttactatgatatccattttccagaattgtgattacaatatgcaaagagtcataaatatgccatttacaataaggaggaggcaaggcaaatgcatagatgtacaaatatatgtacaacagattttgctttttatttatttataatgtaattttatagaataattctgggatttgagaggatctaaaactatttttctgtataaatattatttgccaaaagtttgtttatattcagaagtctgactatgatgaataaatcttaaatgctttgtttaattaaaaaacaaaaatcaccaatatccaagacatgaagatatcagttcaacaaatactgtagttaagagactaactctccacttgtatgggaactacatttcactcttggttttcaggatataacagcacttcaccgaaatattctttcagccataccactggtaacatttctactaaatctttctgtaacacttaaagaattccctcattcattaccttacagtgtaaacaggagtctaatttgtatcaatactatgttttggttgtaatattcagttcactcacccaatgtacaaccaatgaaataaaagaagcatttaaaagg

SEQ ID NO: 56 - DNA, 2783 bp, synthetic construct
  misc_feature 1..2783: note = Insert of plasmid pEZX-MT05 with the 3'UTR of MBNL2 modified to have perfect complementarity with miR-23b (3'UTR Pm-23b)
  misc_feature 646..666: note = /note="Region modified for perfect complementarity with miR23b"
  source 1..2783: mol_type = other DNA
tcagcagaaacggaatggaatgccaagaatctgcattgagaataactaaacattgttactgtacatactatcctgtttcctcctcaatagaattgccacaaactgcatgctaaataaagatgtagttcttctggacagaccacaactctaagaagctagtgctgctatctcatatatgagtattaaatatggtatgcttagtatattccaacctaagatagttaactacctgagaccagctgtgatgtttaaagacataaaggataaagtttacttttaaagggtttctaaacatagtttctgtcctaggaatattgtcttatctccataactatagctgatgcagaaagtccagccagtttactcatttcgattcagaatatttcaaatttagcaataaacaattagcattagttaaaaaagaaacatattccaagggcaggttcgattctagctctaattactgtcatgtcatttacccactggatcaaagggtatgtttcacttcttgacaatataaatgctgcagcaaagatgagaggtgaagtaaaaccgatacctgtcctgcaggtctaaaatttgaatggaaattcaagcacaagtactggggacacatcaaagtgtggtgtttggtttgcctggagaggtaatccctggcaatgtgattctagattaacattaaatagattgaaaaagaaactttgcacggtatgagcttcataccccaccaaacaaagtcttgaaggtattattttacaagtatatttttaaagttgttttataagagagactttgtagaagtgcctagattttgccagacttcatccagcttgacaagattgagaggcccatgccaacagtctaatctaagagattagtctttcaaactcaccatccagttgcctgttacagaataactcttcttaactaaaaacctagtcaaacaaggaagctgtaggtgaggagatctgtataatattctaatttaagtaagtttgagtttagtcactgcaaatttgactgtgactttaatctaaattactatgtaaacaaaaagtagatagtttcactttttaaaaaatccattactgttttgcatttcaaaagttggattaaagggttgtaactgactacagcatggaaaaaaatagttcttttaattctttcaccttaaagcatattttatgtctcaaaagtataaaaaactttaatacaagtacatacatattatatatacacatacatatatatactatatatggatgaaacatattttaatgttgtttacttttttaaatacttggttgatcttcaaggtaatagcgatacaattaaattttgttcagaaagtttgttttaaagtttattttaagcactatcgtaccaaatatttcatatttcacattttatatgttgcacatagcctatacagtacctacatagtttttaaattattgtttaaaaaacaaaacagctgttataaatgaatattatgtgtaattgtttcaaacatccattttctttgtgaacatattagtgattgaagtattttgacttttgagattgaatgtaaaatattttaaatttgggatcatcgcctgttctgaaaactagatgcaccaaccgtatcattatttgtttgaggaaaaaaagaaatctgcattttaattcatgttggtcaaagtcgaattactatctatttatcttatatcgtagatctgataaccctatctaaaagaaagtcacacgctaaatgtattcttacatagtgcttgtatcgttgcatttgttttaatttgtggaaaagtattgtatctaacttgtattactttggtagtttcatctttatgtattattgatatttgtaattttctcaactataacaatgtagttacgctacaacttgcctaaaacattcaaacttgttttcttttttctgtttttttctttgttaattcatttaaactcattgaaaacatagtatacattactaaaaggtaaattatgggaatcactgaaatatttttgtagattaattgttgtaacattgtctttcttttttttcttttgtttcatgattttgatttttaaaattattagcacacaactattttcagccctttaataatggagcatcaaaaacatcacctgtaaccccaagcaaatatagaagactgtattttttactatgatatccattttccagaattgtgattacaatatgcaaagagtcataaatatgccatttacaataaggaggaggcaaggcaaatgcatagatgtacaaatatatgtacaacagattttgctttttatttatttataatgtaattttatagaataattctgggatttgagaggatctaaaactatttttctgtataaatattatttgccaaaagtttgtttatattcagaagtctgactatgatgaataaatcttaaatgctttgtttaattaaaaaacaaaaatcaccaatatccaagacatgaagatatcagttcaacaaatactgtagttaagagactaactctccacttgtatgggaactacatttcactcttggttttcaggatataacagcacttcaccgaaatattctttcagccataccactggtaacatttctactaaatctttctgtaacacttaaagaattccctcattcattaccttacagtgtaaacaggagtctaatttgtatcaatactatgttttggttgtaatattcagttcactcacccaatgtacaaccaatgaaataaaagaagcatttaaaagg

SEQ ID NO: 57 - DNA, 2776 bp, synthetic construct
  misc_feature 1..2776: note = Insert area of plasmid pEZX-MT05 with the 3'UTR of MBNL2 with seed region of miR-218 deleted (3'UTR MUT1-218)
  misc_feature 593..594: note = /note="Flanking nucleotides of the deletion in the seed region of miR-218"
  source 1..2776: mol_type = other DNA
tcagcagaaacggaatggaatgccaagaatctgcattgagaataactaaacattgttactgtacatactatcctgtttcctcctcaatagaattgccacaaactgcatgctaaataaagatgtagttcttctggacagaccacaactctaagaagctagtgctgctatctcatatatgagtattaaatatggtatgcttagtatattccaacctaagatagttaactacctgagaccagctgtgatgtttaaagacataaaggataaagtttacttttaaagggtttctaaacatagtttctgtcctaggaatattgtcttatctccataactatagctgatgcagaaagtccagccagtttactcatttcgattcagaatatttcaaatttagcaataaacaattagcattagttaaaaaagaaacatattccaagggcaggttcgattctagctctaattactgtcatgtcatttacccactggatcaaagggtatgtttcacttcttgacaatataaatgctgcagcaaagatgagaggtgaagtaaaaccgatacctgtcctgcaggtctaaaatttgaatggaaattcagtactggggacacatcaaagtgtggtgtttggtttgcctggagatgccacgttgaatcatgtgattctagattaacattaaatagattgaaaaagaaactttgcacggtatgagcttcataccccaccaaacaaagtcttgaaggtattattttacaagtatatttttaaagttgttttataagagagactttgtagaagtgcctagattttgccagacttcatccagcttgacaagattgagaggcccatgccaacagtctaatctaagagattagtctttcaaactcaccatccagttgcctgttacagaataactcttcttaactaaaaacctagtcaaacaaggaagctgtaggtgaggagatctgtataatattctaatttaagtaagtttgagtttagtcactgcaaatttgactgtgactttaatctaaattactatgtaaacaaaaagtagatagtttcactttttaaaaaatccattactgttttgcatttcaaaagttggattaaagggttgtaactgactacagcatggaaaaaaatagttcttttaattctttcaccttaaagcatattttatgtctcaaaagtataaaaaactttaatacaagtacatacatattatatatacacatacatatatatactatatatggatgaaacatattttaatgttgtttacttttttaaatacttggttgatcttcaaggtaatagcgatacaattaaattttgttcagaaagtttgttttaaagtttattttaagcactatcgtaccaaatatttcatatttcacattttatatgttgcacatagcctatacagtacctacatagtttttaaattattgtttaaaaaacaaaacagctgttataaatgaatattatgtgtaattgtttcaaacatccattttctttgtgaacatattagtgattgaagtattttgacttttgagattgaatgtaaaatattttaaatttgggatcatcgcctgttctgaaaactagatgcaccaaccgtatcattatttgtttgaggaaaaaaagaaatctgcattttaattcatgttggtcaaagtcgaattactatctatttatcttatatcgtagatctgataaccctatctaaaagaaagtcacacgctaaatgtattcttacatagtgcttgtatcgttgcatttgttttaatttgtggaaaagtattgtatctaacttgtattactttggtagtttcatctttatgtattattgatatttgtaattttctcaactataacaatgtagttacgctacaacttgcctaaaacattcaaacttgttttcttttttctgtttttttctttgttaattcatttaaactcattgaaaacatagtatacattactaaaaggtaaattatgggaatcactgaaatatttttgtagattaattgttgtaacattgtctttcttttttttcttttgtttcatgattttgatttttaaaattattagcacacaactattttcagccctttaataatggagcatcaaaaacatcacctgtaaccccaagcaaatatagaagactgtattttttactatgatatccattttccagaattgtgattacaatatgcaaagagtcataaatatgccatttacaataaggaggaggcaaggcaaatgcatagatgtacaaatatatgtacaacagattttgctttttatttatttataatgtaattttatagaataattctgggatttgagaggatctaaaactatttttctgtataaatattatttgccaaaagtttgtttatattcagaagtctgactatgatgaataaatcttaaatgctttgtttaattaaaaaacaaaaatcaccaatatccaagacatgaagatatcagttcaacaaatactgtagttaagagactaactctccacttgtatgggaactacatttcactcttggttttcaggatataacagcacttcaccgaaatattctttcagccataccactggtaacatttctactaaatctttctgtaacacttaaagaattccctcattcattaccttacagtgtaaacaggagtctaatttgtatcaatactatgttttggttgtaatattcagttcactcacccaatgtacaaccaatgaaataaaagaagcatttaaaagg

SEQ ID NO: 58 - DNA, 2776 bp, synthetic construct
  misc_feature 1..2776: note = Insert area of plasmid pEZX-MT05 with the 3'UTR of MBNL2 with seed region of miR-218 deleted (3'UTR MUT1-218)
  misc_feature 1370..1371: note = /note="Flanking nucleotides of the miR-218 binding seed region deleted"
  source 1..2776: mol_type = other DNA
tcagcagaaacggaatggaatgccaagaatctgcattgagaataactaaacattgttactgtacatactatcctgtttcctcctcaatagaattgccacaaactgcatgctaaataaagatgtagttcttctggacagaccacaactctaagaagctagtgctgctatctcatatatgagtattaaatatggtatgcttagtatattccaacctaagatagttaactacctgagaccagctgtgatgtttaaagacataaaggataaagtttacttttaaagggtttctaaacatagtttctgtcctaggaatattgtcttatctccataactatagctgatgcagaaagtccagccagtttactcatttcgattcagaatatttcaaatttagcaataaacaattagcattagttaaaaaagaaacatattccaagggcaggttcgattctagctctaattactgtcatgtcatttacccactggatcaaagggtatgtttcacttcttgacaatataaatgctgcagcaaagatgagaggtgaagtaaaaccgatacctgtcctgcaggtctaaaatttgaatggaaattcaagcacaagtactggggacacatcaaagtgtggtgtttggtttgcctggagatgccacgttgaatcatgtgattctagattaacattaaatagattgaaaaagaaactttgcacggtatgagcttcataccccaccaaacaaagtcttgaaggtattattttacaagtatatttttaaagttgttttataagagagactttgtagaagtgcctagattttgccagacttcatccagcttgacaagattgagaggcccatgccaacagtctaatctaagagattagtctttcaaactcaccatccagttgcctgttacagaataactcttcttaactaaaaacctagtcaaacaaggaagctgtaggtgaggagatctgtataatattctaatttaagtaagtttgagtttagtcactgcaaatttgactgtgactttaatctaaattactatgtaaacaaaaagtagatagtttcactttttaaaaaatccattactgttttgcatttcaaaagttggattaaagggttgtaactgactacagcatggaaaaaaatagttcttttaattctttcaccttaaagcatattttatgtctcaaaagtataaaaaactttaatacaagtacatacatattatatatacacatacatatatatactatatatggatgaaacatattttaatgttgtttacttttttaaatacttggttgatcttcaaggtaatagcgatacaattaaattttgttcagaaagtttgttttaaagtttattttatcgtaccaaatatttcatatttcacattttatatgttgcacatagcctatacagtacctacatagtttttaaattattgtttaaaaaacaaaacagctgttataaatgaatattatgtgtaattgtttcaaacatccattttctttgtgaacatattagtgattgaagtattttgacttttgagattgaatgtaaaatattttaaatttgggatcatcgcctgttctgaaaactagatgcaccaaccgtatcattatttgtttgaggaaaaaaagaaatctgcattttaattcatgttggtcaaagtcgaattactatctatttatcttatatcgtagatctgataaccctatctaaaagaaagtcacacgctaaatgtattcttacatagtgcttgtatcgttgcatttgttttaatttgtggaaaagtattgtatctaacttgtattactttggtagtttcatctttatgtattattgatatttgtaattttctcaactataacaatgtagttacgctacaacttgcctaaaacattcaaacttgttttcttttttctgtttttttctttgttaattcatttaaactcattgaaaacatagtatacattactaaaaggtaaattatgggaatcactgaaatatttttgtagattaattgttgtaacattgtctttcttttttttcttttgtttcatgattttgatttttaaaattattagcacacaactattttcagccctttaataatggagcatcaaaaacatcacctgtaaccccaagcaaatatagaagactgtattttttactatgatatccattttccagaattgtgattacaatatgcaaagagtcataaatatgccatttacaataaggaggaggcaaggcaaatgcatagatgtacaaatatatgtacaacagattttgctttttatttatttataatgtaattttatagaataattctgggatttgagaggatctaaaactatttttctgtataaatattatttgccaaaagtttgtttatattcagaagtctgactatgatgaataaatcttaaatgctttgtttaattaaaaaacaaaaatcaccaatatccaagacatgaagatatcagttcaacaaatactgtagttaagagactaactctccacttgtatgggaactacatttcactcttggttttcaggatataacagcacttcaccgaaatattctttcagccataccactggtaacatttctactaaatctttctgtaacacttaaagaattccctcattcattaccttacagtgtaaacaggagtctaatttgtatcaatactatgttttggttgtaatattcagttcactcacccaatgtacaaccaatgaaataaaagaagcatttaaaagg

SEQ ID NO: 59 - DNA, 2777 bp, synthetic construct
  misc_feature 1..2777: note = Insert area of plasmid pEZX-MT05 with the 3'UTR of MBNL2 with seed region of miR-218 deleted (3'UTR MUT1-218)
  misc_feature 2088..2089: note = /note="Flanking nucleotides of the seed region of mir-218 deleted"
  source 1..2777: mol_type = other DNA
tcagcagaaacggaatggaatgccaagaatctgcattgagaataactaaacattgttactgtacatactatcctgtttcctcctcaatagaattgccacaaactgcatgctaaataaagatgtagttcttctggacagaccacaactctaagaagctagtgctgctatctcatatatgagtattaaatatggtatgcttagtatattccaacctaagatagttaactacctgagaccagctgtgatgtttaaagacataaaggataaagtttacttttaaagggtttctaaacatagtttctgtcctaggaatattgtcttatctccataactatagctgatgcagaaagtccagccagtttactcatttcgattcagaatatttcaaatttagcaataaacaattagcattagttaaaaaagaaacatattccaagggcaggttcgattctagctctaattactgtcatgtcatttacccactggatcaaagggtatgtttcacttcttgacaatataaatgctgcagcaaagatgagaggtgaagtaaaaccgatacctgtcctgcaggtctaaaatttgaatggaaattcaagcacaagtactggggacacatcaaagtgtggtgtttggtttgcctggagatgccacgttgaatcatgtgattctagattaacattaaatagattgaaaaagaaactttgcacggtatgagcttcataccccaccaaacaaagtcttgaaggtattattttacaagtatatttttaaagttgttttataagagagactttgtagaagtgcctagattttgccagacttcatccagcttgacaagattgagaggcccatgccaacagtctaatctaagagattagtctttcaaactcaccatccagttgcctgttacagaataactcttcttaactaaaaacctagtcaaacaaggaagctgtaggtgaggagatctgtataatattctaatttaagtaagtttgagtttagtcactgcaaatttgactgtgactttaatctaaattactatgtaaacaaaaagtagatagtttcactttttaaaaaatccattactgttttgcatttcaaaagttggattaaagggttgtaactgactacagcatggaaaaaaatagttcttttaattctttcaccttaaagcatattttatgtctcaaaagtataaaaaactttaatacaagtacatacatattatatatacacatacatatatatactatatatggatgaaacatattttaatgttgtttacttttttaaatacttggttgatcttcaaggtaatagcgatacaattaaattttgttcagaaagtttgttttaaagtttattttaagcactatcgtaccaaatatttcatatttcacattttatatgttgcacatagcctatacagtacctacatagtttttaaattattgtttaaaaaacaaaacagctgttataaatgaatattatgtgtaattgtttcaaacatccattttctttgtgaacatattagtgattgaagtattttgacttttgagattgaatgtaaaatattttaaatttgggatcatcgcctgttctgaaaactagatgcaccaaccgtatcattatttgtttgaggaaaaaaagaaatctgcattttaattcatgttggtcaaagtcgaattactatctatttatcttatatcgtagatctgataaccctatctaaaagaaagtcacacgctaaatgtattcttacatagtgcttgtatcgttgcatttgttttaatttgtggaaaagtattgtatctaacttgtattactttggtagtttcatctttatgtattattgatatttgtaattttctcaactataacaatgtagttacgctacaacttgcctaaaacattcaaacttgttttcttttttctgtttttttctttgttaattcatttaaactcattgaaaacatagtatacattactaaaaggtaaattatgggaatcactgaaatatttttgtagattaattgttgtaacattgtctttcttttttttcttttgtttcatgattttgatttttaaaattattcaactattttcagccctttaataatggagcatcaaaaacatcacctgtaaccccaagcaaatatagaagactgtattttttactatgatatccattttccagaattgtgattacaatatgcaaagagtcataaatatgccatttacaataaggaggaggcaaggcaaatgcatagatgtacaaatatatgtacaacagattttgctttttatttatttataatgtaattttatagaataattctgggatttgagaggatctaaaactatttttctgtataaatattatttgccaaaagtttgtttatattcagaagtctgactatgatgaataaatcttaaatgctttgtttaattaaaaaacaaaaatcaccaatatccaagacatgaagatatcagttcaacaaatactgtagttaagagactaactctccacttgtatgggaactacatttcactcttggttttcaggatataacagcacttcaccgaaatattctttcagccataccactggtaacatttctactaaatctttctgtaacacttaaagaattccctcattcattaccttacagtgtaaacaggagtctaatttgtatcaatactatgttttggttgtaatattcagttcactcacccaatgtacaaccaatgaaataaaagaagcatttaaaagg

SEQ ID NO: 60 - DNA, 2784 bp, synthetic construct
  misc_feature 1..2784: note = Insert of plasmid pEZX-MT05 with the 3'UTR of MBNL2 modified to have perfect complementarity with miR-23b (3'UTR PM-2218)
  misc_feature 582..602: note = /note="Region modified for perfect complementarity with miR-218"
  misc_feature 1359..1379: note = /note="Region modified for perfect complementarity with miR-218"
  misc_feature 2086..2106: note = /note="Region modified for perfect complementarity with miR-218"
  source 1..2784: mol_type = other DNA
tcagcagaaacggaatggaatgccaagaatctgcattgagaataactaaacattgttactgtacatactatcctgtttcctcctcaatagaattgccacaaactgcatgctaaataaagatgtagttcttctggacagaccacaactctaagaagctagtgctgctatctcatatatgagtattaaatatggtatgcttagtatattccaacctaagatagttaactacctgagaccagctgtgatgtttaaagacataaaggataaagtttacttttaaagggtttctaaacatagtttctgtcctaggaatattgtcttatctccataactatagctgatgcagaaagtccagccagtttactcatttcgattcagaatatttcaaatttagcaataaacaattagcattagttaaaaaagaaacatattccaagggcaggttcgattctagctctaattactgtcatgtcatttacccactggatcaaagggtatgtttcacttcttgacaatataaatgctgcagcaaagatgagaggtgaagtaaaaccgatacctgtcctgcaggtctaaaatttacatggttagatcaagcacaagtactggggacacatcaaagtgtggtgtttggtttgcctggagatgccacgttgaatcatgtgattctagattaacattaaatagattgaaaaagaaactttgcacggtatgagcttcataccccaccaaacaaagtcttgaaggtattattttacaagtatatttttaaagttgttttataagagagactttgtagaagtgcctagattttgccagacttcatccagcttgacaagattgagaggcccatgccaacagtctaatctaagagattagtctttcaaactcaccatccagttgcctgttacagaataactcttcttaactaaaaacctagtcaaacaaggaagctgtaggtgaggagatctgtataatattctaatttaagtaagtttgagtttagtcactgcaaatttgactgtgactttaatctaaattactatgtaaacaaaaagtagatagtttcactttttaaaaaatccattactgttttgcatttcaaaagttggattaaagggttgtaactgactacagcatggaaaaaaatagttcttttaattctttcaccttaaagcatattttatgtctcaaaagtataaaaaactttaatacaagtacatacatattatatatacacatacatatatatactatatatggatgaaacatattttaatgttgtttacttttttaaatacttggttgatcttcaaggtaatagcgatacaattaaattttgttcagaaagtttgtttacatggttagatcaagcacaatcgtaccaaatatttcatatttcacattttatatgttgcacatagcctatacagtacctacatagtttttaaattattgtttaaaaaacaaaacagctgttataaatgaatattatgtgtaattgtttcaaacatccattttctttgtgaacatattagtgattgaagtattttgacttttgagattgaatgtaaaatattttaaatttgggatcatcgcctgttctgaaaactagatgcaccaaccgtatcattatttgtttgaggaaaaaaagaaatctgcattttaattcatgttggtcaaagtcgaattactatctatttatcttatatcgtagatctgataaccctatctaaaagaaagtcacacgctaaatgtattcttacatagtgcttgtatcgttgcatttgttttaatttgtggaaaagtattgtatctaacttgtattactttggtagtttcatctttatgtattattgatatttgtaattttctcaactataacaatgtagttacgctacaacttgcctaaaacattcaaacttgttttcttttttctgtttttttctttgttaattcatttaaactcattgaaaacatagtatacattactaaaaggtaaattatgggaatcactgaaatatttttgtagattaattgttgtaacattgtctttcttttttttcttttgtttcatgattttgaacatggttagatcaagcacaaaactattttcagccctttaataatggagcatcaaaaacatcacctgtaaccccaagcaaatatagaagactgtattttttactatgatatccattttccagaattgtgattacaatatgcaaagagtcataaatatgccatttacaataaggaggaggcaaggcaaatgcatagatgtacaaatatatgtacaacagattttgctttttatttatttataatgtaattttatagaataattctgggatttgagaggatctaaaactatttttctgtataaatattatttgccaaaagtttgtttatattcagaagtctgactatgatgaataaatcttaaatgctttgtttaattaaaaaacaaaaatcaccaatatccaagacatgaagatatcagttcaacaaatactgtagttaagagactaactctccacttgtatgggaactacatttcactcttggttttcaggatataacagcacttcaccgaaatattctttcagccataccactggtaacatttctactaaatctttctgtaacacttaaagaattccctcattcattaccttacagtgtaaacaggagtctaatttgtatcaatactatgttttggttgtaatattcagttcactcacccaatgtacaaccaatgaaataaaagaagcatttaaaagg

SEQ ID NO: 61 - DNA, 20 bp, synthetic construct
  misc_feature 1..20: note = Probe for the detection of foci in thorax of flies (CAG probe)
  misc_feature 1: note = /note="Fluorophore Cy3 bound at 5'"
  misc_feature 20: note = /note="Fluorophore Cy3 bound at 3'"
  source 1..20: mol_type = other DNA
cagcagcagcagcagcagca

SEQ ID NO: 62 - DNA, 496 bp, synthetic construct
  misc_feature 1..496: note = Sequence of the fragment of sponge construct with 20 repeat targets for DME-miR-92a
  misc_feature 1..21: note = /note="Target of microRNA dme-miR-92a"
  misc_feature 22..25: note = /note="Spacer fragment"
  misc_feature 26..46: note = /note="Target of microRNA dme-miR-92a"
  misc_feature 47..50: note = /note="Spacer fragment"
  misc_feature 51..71: note = /note="Target of microRNA dme-miR-92a"
  misc_feature 72..75: note = /note="Spacer fragment"
  misc_feature 76..96: note = /note="Target of microRNA dme-miR-92a"
  misc_feature 97..100: note = /note="Spacer fragment"
  misc_feature 101..121: note = /note="Target of microRNA dme-miR-92a"
  misc_feature 122..125: note = /note="Spacer fragment"
  misc_feature 126..146: note = /note="Target of microRNA dme-miR-92a"
  misc_feature 147..150: note = /note="Spacer fragment"
  misc_feature 151..171: note = /note="Target of microRNA dme-miR-92a"
  misc_feature 172..175: note = /note="Spacer fragment"
  misc_feature 176..196: note = /note="Target of microRNA dme-miR-92a"
  misc_feature 197..200: note = /note="Spacer fragment"
  misc_feature 201..221: note = /note="Target of microRNA dme-miR-92a"
  misc_feature 222..225: note = /note="Spacer fragment"
  misc_feature 226..246: note = /note="Target of microRNA dme-miR-92a"
  misc_feature 247..250: note = /note="Spacer fragment"
  misc_feature 251..271: note = /note="Target of microRNA dme-miR-92a"
  misc_feature 272..275: note = /note="Spacer fragment"
  misc_feature 276..296: note = /note="Target of microRNA dme-miR-92a"
  misc_feature 297..300: note = /note="Spacer fragment"
  misc_feature 301..321: note = /note="Target of microRNA dme-miR-92a"
  misc_feature 322..325: note = /note="Spacer fragment"
  misc_feature 326..346: note = /note="Target of microRNA dme-miR-92a"
  misc_feature 347..350: note = /note="Spacer fragment"
  misc_feature 351..371: note = /note="Target of microRNA dme-miR-92a"
  misc_feature 372..375: note = /note="Spacer fragment"
  misc_feature 376..396: note = /note="Target of microRNA dme-miR-92a"
  misc_feature 397..400: note = /note="Spacer fragment"
  misc_feature 401..421: note = /note="Target of microRNA dme-miR-92a"
  misc_feature 422..425: note = /note="Spacer fragment"
  misc_feature 426..446: note = /note="Target of microRNA dme-miR-92a"
  misc_feature 447..450: note = /note="Spacer fragment"
  misc_feature 451..471: note = /note="Target of microRNA dme-miR-92a"
  misc_feature 472..475: note = /note="Spacer fragment"
  misc_feature 476..496: note = /note="Target of microRNA dme-miR-92a"
  source 1..496: mol_type = other DNA
ataggccggggttgtgcaatggcgcataggccggggttgtgcaatgggccataggccggggttgtgcaatgggctataggccggggttgtgcaatgggggataggccggggttgtgcaatgggatataggccggggttgtgcaatgggtcataggccggggttgtgcaatgggtgataggccggggttgtgcaatgggttataggccggggttgtgcaatggaccataggccggggttgtgcaatgggtgataggccggggttgtgcaatggcgcataggccggggttgtgcaatgggccataggccggggttgtgcaatgggctataggccggggttgtgcaatgggggataggccggggttgtgcaatgggatataggccggggttgtgcaatgggtcataggccggggttgtgcaatgggtgataggccggggttgtgcaatgggttataggccggggttgtgcaatggaccataggccggggttgtgcaatg

SEQ ID NO: 63 - DNA, 496 bp, synthetic construct
  misc_feature 1..496: note = Sequence of the fragment of sponge construct with 20 repeat targets for dme-miR-100
  misc_feature 1..21: note = /note="Target of microRNA dme-miR-100"
  misc_feature 22..25: note = /note="Spacer fragment"
  misc_feature 26..46: note = /note="Target of microRNA dme-miR-100"
  misc_feature 47..50: note = /note="Spacer fragment"
  misc_feature 51..71: note = /note="Target of microRNA dme-miR-100"
  misc_feature 72..75: note = /note="Spacer fragment"
  misc_feature 76..96: note = /note="Target of microRNA dme-miR-100"
  misc_feature 97..100: note = /note="Spacer fragment"
  misc_feature 101..121: note = /note="Target of microRNA dme-miR-100"
  misc_feature 122..125: note = /note="Spacer fragment"
  misc_feature 126..146: note = /note="Target of microRNA dme-miR-100"
  misc_feature 147..150: note = /note="Spacer fragment"
  misc_feature 151..171: note = /note="Target of microRNA dme-miR-100"
  misc_feature 172..175: note = /note="Spacer fragment"
  misc_feature 176..196: note = /note="Target of microRNA dme-miR-100"
  misc_feature 197..200: note = /note="Spacer fragment"
  misc_feature 201..221: note = /note="Target of microRNA dme-miR-100"
  misc_feature 222..225: note = /note="Spacer fragment"
  misc_feature 226..246: note = /note="Target of microRNA dme-miR-100"
  misc_feature 247..250: note = /note="Spacer fragment"
  misc_feature 251..271: note = /note="Target of microRNA dme-miR-100"
  misc_feature 272..275: note = /note="Spacer fragment"
  misc_feature 276..296: note = /note="Target of microRNA dme-miR-100"
  misc_feature 297..300: note = /note="Spacer fragment"
  misc_feature 301..321: note = /note="Target of microRNA dme-miR-100"
  misc_feature 322..325: note = /note="Spacer fragment"
  misc_feature 326..346: note = /note="Target of microRNA dme-miR-100"
  misc_feature 347..350: note = /note="Spacer fragment"
  misc_feature 351..371: note = /note="Target of microRNA dme-miR-100"
  misc_feature 372..375: note = /note="Spacer fragment"
  misc_feature 376..396: note = /note="Target of microRNA dme-miR-100"
  misc_feature 397..400: note = /note="Spacer fragment"
  misc_feature 401..421: note = /note="Target of microRNA dme-miR-100"
  misc_feature 422..425: note = /note="Spacer fragment"
  misc_feature 426..446: note = /note="Target of microRNA dme-miR-100"
  misc_feature 447..450: note = /note="Spacer fragment"
  misc_feature 451..471: note = /note="Target of microRNA dme-miR-100"
  misc_feature 472..475: note = /note="Spacer fragment"
  misc_feature 476..496: note = /note="Target of microRNA dme-miR-100"
  source 1..496: mol_type = other DNA
cacaagttcgtaatacgggttccgccacaagttcgtaatacgggttccggcacaagttcgtaatacgggttcctccacaagttcgtaatacgggttcctgcacaagttcgtaatacgggttcggacacaagttcgtaatacgggttcgaccacaagttcgtaatacgggttcgtacacaagttcgtaatacgggttctgccacaagttcgtaatacgggttctggcacaagttcgtaatacgggttcgaccacaagttcgtaatacgggttccgccacaagttcgtaatacgggttccggcacaagttcgtaatacgggttcctccacaagttcgtaatacgggttcctgcacaagttcgtaatacgggttcggacacaagttcgtaatacgggttcgaccacaagttcgtaatacgggttcgtacacaagttcgtaatacgggttctgccacaagttcgtaatacgggttctggcacaagttcgtaatacgggtt

SEQ ID NO: 64 - DNA, 516 bp, synthetic construct
  misc_feature 1..516: note = Sequence of the fragment of sponge construct with 20 repeat targets for dme-miR-124
  misc_feature 1..22: note = /note="Sequence of target of microRNA dme-miR-124"
  misc_feature 23..26: note = /note="Spacer fragment"
  misc_feature 27..48: note = /note="Sequence of target of microRNA dme-miR-124"
  misc_feature 49..52: note = /note="Spacer fragment"
  misc_feature 53..74: note = /note="Sequence of target of microRNA dme-miR-124"
  misc_feature 75..78: note = /note="Spacer fragment"
  misc_feature 79..100: note = /note="Sequence of target of microRNA dme-miR-124"
  misc_feature 101..104: note = /note="Spacer fragment"
  misc_feature 105..126: note = /note="Sequence of target of microRNA dme-miR-124"
  misc_feature 127..130: note = /note="Spacer fragment"
  misc_feature 131..152: note = /note="Sequence of target of microRNA dme-miR-124"
  misc_feature 153..156: note = /note="Spacer fragment"
  misc_feature 157..178: note = /note="Sequence of target of microRNA dme-miR-124"
  misc_feature 179..182: note = /note="Spacer fragment"
  misc_feature 183..204: note = /note="Sequence of target of microRNA dme-miR-124"
  misc_feature 205..208: note = /note="Spacer fragment"
  misc_feature 209..230: note = /note="Sequence of target of microRNA dme-miR-124"
  misc_feature 231..234: note = /note="Spacer fragment"
  misc_feature 235..256: note = /note="Sequence of target of microRNA dme-miR-124"
  misc_feature 257..260: note = /note="Spacer fragment"
  misc_feature 261..282: note = /note="Sequence of target of microRNA dme-miR-124"
  misc_feature 283..286: note = /note="Spacer fragment"
  misc_feature 287..308: note = /note="Sequence of target of microRNA dme-miR-124"
  misc_feature 309..312: note = /note="Spacer fragment"
  misc_feature 313..334: note = /note="Sequence of target of microRNA dme-miR-124"
  misc_feature 335..338: note = /note="Spacer fragment"
  misc_feature 339..360: note = /note="Sequence of target of microRNA dme-miR-124"
  misc_feature 361..364: note = /note="Spacer fragment"
  misc_feature 365..386: note = /note="Sequence of target of microRNA dme-miR-124"
  misc_feature 387..390: note = /note="Spacer fragment"
  misc_feature 391..412: note = /note="Sequence of target of microRNA dme-miR-124"
  misc_feature 413..416: note = /note="Spacer fragment"
  misc_feature 417..438: note = /note="Sequence of target of microRNA dme-miR-124"
  misc_feature 439..442: note = /note="Spacer fragment"
  misc_feature 443..464: note = /note="Sequence of target of microRNA dme-miR-124"
  misc_feature 465..468: note = /note="Spacer fragment"
  misc_feature 469..490: note = /note="Sequence of target of microRNA dme-miR-124"
  misc_feature 491..494: note = /note="Spacer fragment"
  misc_feature 495..516: note = /note="Sequence of target of microRNA dme-miR-124"
  source 1..516: mol_type = other DNA
cttggcattcagcggtgccttaccctcttggcattcagcggtgccttaccgccttggcattcagcggtgccttaccggcttggcattcagcggtgccttaccgacttggcattcagcggtgccttaccgtcttggcattcagcggtgccttacgcgcttggcattcagcggtgccttacgctcttggcattcagcggtgccttacggacttggcattcagcggtgccttacggtcttggcattcagcggtgccttaccgacttggcattcagcggtgccttaccctcttggcattcagcggtgccttaccgccttggcattcagcggtgccttaccggcttggcattcagcggtgccttaccgacttggcattcagcggtgccttaccgtcttggcattcagcggtgccttacgcgcttggcattcagcggtgccttacgctcttggcattcagcggtgccttacggacttggcattcagcggtgccttacggtcttggcattcagcggtgcctta

SEQ ID NO: 65 - DNA, 516 bp, synthetic construct
  misc_feature 1..516: note = Sequence of the fragment of sponge construct with 20 repeat targets for dme-miR-277
  misc_feature 1..22: note = /note="Sequence of target of microRNA dme-miR-277"
  misc_feature 23..26: note = /note="Spacer fragment"
  misc_feature 27..48: note = /note="Sequence of target of microRNA dme-miR-277"
  misc_feature 49..52: note = /note="Spacer fragment"
  misc_feature 53..74: note = /note="Sequence of target of microRNA dme-miR-277"
  misc_feature 75..78: note = /note="Spacer fragment"
  misc_feature 79..100: note = /note="Sequence of target of microRNA dme-miR-277"
  misc_feature 101..104: note = /note="Spacer fragment"
  misc_feature 105..126: note = /note="Sequence of target of microRNA dme-miR-277"
  misc_feature 127..130: note = /note="Spacer fragment"
  misc_feature 131..152: note = /note="Sequence of target of microRNA dme-miR-277"
  misc_feature 153..156: note = /note="Spacer fragment"
  misc_feature 157..178: note = /note="Sequence of target of microRNA dme-miR-277"
  misc_feature 179..182: note = /note="Spacer fragment"
  misc_feature 183..204: note = /note="Sequence of target of microRNA dme-miR-277"
  misc_feature 205..208: note = /note="Spacer fragment"
  misc_feature 209..230: note = /note="Sequence of target of microRNA dme-miR-277"
  misc_feature 231..234: note = /note="Spacer fragment"
  misc_feature 235..256: note = /note="Sequence of target of microRNA dme-miR-277"
  misc_feature 257..260: note = /note="Spacer fragment"
  misc_feature 261..282: note = /note="Sequence of target of microRNA dme-miR-277"
  misc_feature 283..286: note = /note="Spacer fragment"
  misc_feature 287..308: note = /note="Sequence of target of microRNA dme-miR-277"
  misc_feature 309..312: note = /note="Spacer fragment"
  misc_feature 313..334: note = /note="Sequence of target of microRNA dme-miR-277"
  misc_feature 335..338: note = /note="Spacer fragment"
  misc_feature 339..360: note = /note="Sequence of target of microRNA dme-miR-277"
  misc_feature 361..364: note = /note="Spacer fragment"
  misc_feature 365..386: note = /note="Sequence of target of microRNA dme-miR-277"
  misc_feature 387..390: note = /note="Spacer fragment"
  misc_feature 391..412: note = /note="Sequence of target of microRNA dme-miR-277"
  misc_feature 413..416: note = /note="Spacer fragment"
  misc_feature 417..438: note = /note="Sequence of target of microRNA dme-miR-277"
  misc_feature 439..442: note = /note="Spacer fragment"
  misc_feature 443..464: note = /note="Sequence of target of microRNA dme-miR-277"
  misc_feature 465..468: note = /note="Spacer fragment"
  misc_feature 469..490: note = /note="Sequence of target of microRNA dme-miR-277"
  misc_feature 491..494: note = /note="Spacer fragment"
  misc_feature 495..516: note = /note="Sequence of target of microRNA dme-miR-277"
  source 1..516: mol_type = other DNA
tgtcgtaccagatctgcatttagccctgtcgtaccagatctgcatttagcggtgtcgtaccagatctgcatttagcaatgtcgtaccagatctgcatttagacctgtcgtaccagatctgcatttagacgtgtcgtaccagatctgcatttagatctgtcgtaccagatctgcatttagatgtgtcgtaccagatctgcatttagtcgtgtcgtaccagatctgcatttagtaatgtcgtaccagatctgcatttagatgtgtcgtaccagatctgcatttagccctgtcgtaccagatctgcatttagcggtgtcgtaccagatctgcatttagcaatgtcgtaccagatctgcatttagacctgtcgtaccagatctgcatttagacgtgtcgtaccagatctgcatttagatctgtcgtaccagatctgcatttagatgtgtcgtaccagatctgcatttagtcgtgtcgtaccagatctgcatttagtaatgtcgtaccagatctgcattta

SEQ ID NO: 66 - DNA, 516 bp, synthetic construct
  misc_feature 1..516: note = Sequence of the fragment of sponge construct with 20 repeat targets for dme-miR-304
  misc_feature 1..22: note = /note="Sequence of target of microRNA dme-miR-304"
  misc_feature 23..26: note = /note="Spacer fragment"
  misc_feature 27..48: note = /note="Sequence of target of microRNA dme-miR-304"
  misc_feature 49..52: note = /note="Spacer fragment"
  misc_feature 53..74: note = /note="Sequence of target of microRNA dme-miR-304"
  misc_feature 75..78: note = /note="Spacer fragment"
  misc_feature 79..100: note = /note="Sequence of target of microRNA dme-miR-304"
  misc_feature 101..104: note = /note="Spacer fragment"
  misc_feature 105..126: note = /note="Sequence of target of microRNA dme-miR-304"
  misc_feature 127..130: note = /note="Spacer fragment"
  misc_feature 131..152: note = /note="Sequence of target of microRNA dme-miR-304"
  misc_feature 153..156: note = /note="Spacer fragment"
  misc_feature 157..178: note = /note="Sequence of target of microRNA dme-miR-304"
  misc_feature 179..182: note = /note="Spacer fragment"
  misc_feature 183..204: note = /note="Sequence of target of microRNA dme-miR-304"
  misc_feature 205..208: note = /note="Spacer fragment"
  misc_feature 209..230: note = /note="Sequence of target of microRNA dme-miR-304"
  misc_feature 231..234: note = /note="Spacer fragment"
  misc_feature 235..256: note = /note="Sequence of target of microRNA dme-miR-304"
  misc_feature 257..260: note = /note="Spacer fragment"
  misc_feature 261..282: note = /note="Sequence of target of microRNA dme-miR-304"
  misc_feature 283..286: note = /note="Spacer fragment"
  misc_feature 287..308: note = /note="Sequence of target of microRNA dme-miR-304"
  misc_feature 309..312: note = /note="Spacer fragment"
  misc_feature 313..334: note = /note="Sequence of target of microRNA dme-miR-304"
  misc_feature 335..338: note = /note="Spacer fragment"
  misc_feature 339..360: note = /note="Sequence of target of microRNA dme-miR-304"
  misc_feature 361..364: note = /note="Spacer fragment"
  misc_feature 365..386: note = /note="Sequence of target of microRNA dme-miR-304"
  misc_feature 387..390: note = /note="Spacer fragment"
  misc_feature 391..412: note = /note="Sequence of target of microRNA dme-miR-304"
  misc_feature 413..416: note = /note="Spacer fragment"
  misc_feature 417..438: note = /note="Sequence of target of microRNA dme-miR-304"
  misc_feature 439..442: note = /note="Spacer fragment"
  misc_feature 443..464: note = /note="Sequence of target of microRNA dme-miR-304"
  misc_feature 465..468: note = /note="Spacer fragment"
  misc_feature 469..490: note = /note="Sequence of target of microRNA dme-miR-304"
  misc_feature 491..494: note = /note="Spacer fragment"
  misc_feature 495..516: note = /note="Sequence of target of microRNA dme-miR-304"
  source 1..516: mol_type = other DNA
ctcacatttacttatgagattagcgactcacatttacttatgagattagcagctcacatttacttatgagattagctactcacatttacttatgagattaggcgctcacatttacttatgagattaggcactcacatttacttatgagattaggggctcacatttacttatgagattaggagctcacatttacttatgagattaaccgctcacatttacttatgagattaacggctcacatttacttatgagattaggagctcacatttacttatgagattagcgactcacatttacttatgagattagcagctcacatttacttatgagattagctactcacatttacttatgagattaggcgctcacatttacttatgagattaggcactcacatttacttatgagattaggggctcacatttacttatgagattaggagctcacatttacttatgagattaaccgctcacatttacttatgagattaacggctcacatttacttatgagatta

SEQ ID NO: 67 - DNA, 21 bp, synthetic construct
  misc_feature 1..21: note = Forward primer of gene PCR transcript amplification DLG1
  source 1..21: mol_type = other DNA
agcccgattaaaaaacagtga

SEQ ID NO: 68 - DNA, 22 bp, synthetic construct
  misc_feature 1..22: note = Reverse primer of gene PCR transcript amplification DLG1
  source 1..22: mol_type = other DNA
cgtattcttcttcgaccacggt

SEQ ID NO: 69 - DNA, 23 bp, synthetic construct
  misc_feature 1..23: note = Forward primer of gene PCR transcript amplification CAPZB
  source 1..23: mol_type = other DNA
ggagaaggatgaaactgtgagtg

SEQ ID NO: 70 - DNA, 21 bp, synthetic construct
  misc_feature 1..21: note = Reverse primer of gene PCR transcript amplification CAPZB
  source 1..21: mol_type = other DNA
cagaggtttagcattgctgct

SEQ ID NO: 71 - DNA, 23 bp, synthetic construct
  misc_feature 1..23: note = Forward primer of gene PCR transcript amplification Atp2a1
  source 1..23: mol_type = other DNA
gctcatggtcctcaagatctcac

SEQ ID NO: 72 - DNA, 20 bp, synthetic construct
  misc_feature 1..20: note = Reverse primer of gene PCR transcript amplification Atp2a1
  source 1..20: mol_type = other DNA
gggtcagtgcctcagctttg

SEQ ID NO: 73 - DNA, 21 bp, synthetic construct
  misc_feature 1..21: note = Forward primer of gene PCR transcript amplification Clcn1
  source 1..21: mol_type = other DNA
gtcctcagcaagtttatgtcc

SEQ ID NO: 74 - DNA, 20 bp, synthetic construct
  misc_feature 1..20: note = Reverse primer of gene PCR transcript amplification Clcn1
  source 1..20: mol_type = other DNA
gaatcctcgccagtaattcc

SEQ ID NO: 75 - DNA, 20 bp, synthetic construct
  misc_feature 1..20: note = Forward primer of gene PCR transcript amplification Nfix
  source 1..20: mol_type = other DNA
tcgacgacagtgagatggag

SEQ ID NO: 76 - DNA, 20 bp, synthetic construct
  misc_feature 1..20: note = Reverse primer of gene PCR transcript amplification Nfix
  source 1..20: mol_type = other DNA
caaactccttcagcgagtcc

SEQ ID NO: 77 - DNA, 24 bp, synthetic construct
  misc_feature 1..24: note = Forward primer of gene PCR transcript amplification Capzb
  source 1..24: mol_type = other DNA
gcacgctgaatgagatctactttg

SEQ ID NO: 78 - DNA, 20 bp, synthetic construct
  misc_feature 1..20: note = Reverse primer of gene PCR transcript amplification Capzb
  source 1..20: mol_type = other DNA
ccggttagcgtgaagcagag

SEQ ID NO: 79 - DNA, 20 bp, synthetic construct
  misc_feature 1..20: note = Forward primer of gene PCR transcript amplification of mouse Gapdh
  source 1..20: mol_type = other DNA
atcaacgggaagcccatcac

SEQ ID NO: 80 - DNA, 21 bp, synthetic construct
  misc_feature 1..21: note = Reverse primer of gene PCR transcript amplification of mouse Gapdh
  source 1..21: mol_type = other DNA
cttccacaatgccaaagttgt

SEQ ID NO: 81 - RNA, 97 nt, Homo sapiens
  misc_feature 1..97: note = /note="pre-miRNA of hsa-mir-23b-3p"
  source 1..97: mol_type = other RNA
ctcaggtgctctggctgcttgggttcctggcatgctgatttgtgacttaagattaaaatcacattgccagggattaccacgcaaccacgaccttggc

SEQ ID NO: 82 - RNA, 110 nt, Homo sapiens
  misc_feature 1..110: note = /note="pre-miRNA-1 of hsa-mir-218"
  source 1..110: mol_type = other RNA
gtgataatgtagcgagattttctgttgtgcttgatctaaccatgtggttgcgaggtatgagtaaaacatggttccgtcaagcaccatggaacgtcacgcagctttctaca

SEQ ID NO: 83 - RNA, 110 nt, Homo sapiens
  misc_feature 1..110: note = /note="pre-miRNA-2 of hsa-mir-218"
  source 1..110: mol_type = other RNA
gaccagtcgctgcggggctttcctttgtgcttgatctaaccatgtggtggaacgatggaaacggaacatggttctgtcaagcaccgcggaaagcaccgtgctctcctgca

SEQ ID NO: 84 - RNA, 16 nt, synthetic construct
  modified_base 1: mod_base = OTHER; note = thymine
  modified_base 11..12: mod_base = OTHER; note = thymine
  modified_base 14..16: mod_base = OTHER; note = thymine
  misc_feature 1..16: note = Antagonist MbloCKnoMIR
  misc_feature 1..2: note = /note="LNA nucleotide"
  misc_feature 1..15: note = /note="Phosphorothioate bond"
  misc_feature 3..10: note = /note="2'-O-methyl-nucleotide"
  misc_feature 11..16: note = /note="LNA nucleotide"
  source 1..16: mol_type = other RNA
tgcacctttgttattt

SEQ ID NO: 85 - RNA, 16 nt, synthetic construct
  modified_base 4..5: mod_base = OTHER; note = thymine
  modified_base 15: mod_base = OTHER; note = thymine
  misc_feature 1..16: note = Antagonist MlbloCK23-1
  misc_feature 1..15: note = /note="Phosphorothioate bond"
  misc_feature 7..14: note = /note="2'-O-methyl-nucleotide"
  misc_feature 15..16: note = /note="LNA nucleotide"
  source 1..16: mol_type = other RNA
ccattatcacattttg

SEQ ID NO: 86 - RNA, 16 nt, synthetic construct
  modified_base 10..11: mod_base = OTHER; note = thymine
  misc_feature 1..16: note = Antagonist M2bloCK23-1
  misc_feature 1: note = /note="LNA nucleotide"
  misc_feature 1..14: note = /note="Phosphorothioate bond"
  misc_feature 2..8: note = /note="2'-O-methyl-nucleotide"
  misc_feature 9..15: note = /note="LNA nucleotide"
  source 1..16: mol_type = other RNA
atcacatgattcaacg

SEQ ID NO: 87 - RNA, 16 nt, synthetic construct
  modified_base 14: mod_base = OTHER; note = thymine
  modified_base 16: mod_base = OTHER; note = thymine
  misc_feature 1..16: note = /note="combined DNA/RNA molecule" /note="Antagonist MlbloCK218-1"
  misc_feature 1..2: note = /note="LNA nucleotide"
  misc_feature 1..15: note = /note="Phosphorothioate bond"
  misc_feature 3..10: note = /note="2'-O-methyl-nucleotide"
  misc_feature 11..16: note = /note="LNA nucleotide"
  source 1..16: mol_type = other RNA
gatgtgctttaaatat

SEQ ID NO: 88 - RNA, 16 nt, synthetic construct
  modified_base 10: mod_base = OTHER; note = thymine
  modified_base 12: mod_base = OTHER; note = thymine
  modified_base 14..15: mod_base = OTHER; note = thymine
  misc_feature 1..16: note = /note="combined DNA/RNA molecule" /note="Antagonist MlbloCK218-2"
  misc_feature 1: note = /note="LNA nucleotide"
  misc_feature 1..15: note = /note="Phosphorothioate bond"
  misc_feature 2..9: note = /note="2'-O-methyl-nucleotide"
  misc_feature 10..16: note = /note="LNA nucleotide"
  source 1..16: mol_type = other RNA
gttgtgctgtctattg

SEQ ID NO: 89 - RNA, 16 nt, synthetic construct
  modified_base 3: mod_base = OTHER; note = thymine
  modified_base 15..16: mod_base = OTHER; note = thymine
  misc_feature 1..16: note = /note="combined DNA/RNA molecule" /note="Antagonist M2bloCK218-1"
  misc_feature 1..3: note = /note="LNA nucleotide"
  misc_feature 1..15: note = /note="Phosphorothioate bond"
  misc_feature 4..10: note = /note="2'-O-methyl-nucleotide"
  misc_feature 11..16: note = /note="LNA nucleotide"
  misc_feature 14: note = /note="2'-O-methyl-nucleotide"
  source 1..16: mol_type = other RNA
acttgtgcttgaattt

SEQ ID NO: 90 - RNA, 16 nt, synthetic construct
  modified_base 2..3: mod_base = OTHER; note = thymine
  modified_base 13: mod_base = OTHER; note = thymine
  modified_base 16: mod_base = OTHER; note = thymine
  misc_feature 1..16: note = /note="combined DNA/RNA molecule" /note="Antagonist M2bloCK218-2"
  misc_feature 1..4: note = /note="LNA nucleotide"
  misc_feature 1..15: note = /note="Phosphorothioate bond"
  misc_feature 5..11: note = /note="2'-O-methyl-nucleotide"
  misc_feature 12..16: note = /note="LNA nucleotide"
  source 1..16: mol_type = other RNA
gttgtgtgctaataat

SEQ ID NO: 91 - RNA, 15 nt, synthetic construct
  modified_base 4: mod_base = OTHER; note = thymine
  misc_feature 1..15: note = /note="combined DNA/RNA molecule" /note="Antagonist M2bloCK218-3"
  misc_feature 1..5: note = /note="LNA nucleotide"
  misc_feature 1..14: note = /note="Phosphorothioate bond"
  misc_feature 6..11: note = /note="2'-O-methyl-nucleotide"
  misc_feature 12..15: note = /note="LNA nucleotide"
  source 1..15: mol_type = other RNA
cgatagtgcttaaaa

SEQ ID NO: 92 - RNA, 15 nt, synthetic construct
  modified_base 15: mod_base = OTHER; note = thymine
  misc_feature 1..15: note = /note="combined DNA/RNA molecule" /note="Antagonist AntimiR-23b"
  misc_feature 1..14: note = /note="Phosphorothioate bond"
  misc_feature 1: note = /note="LNA nucleotide"
  misc_feature 7: note = /note="LNA nucleotide"
  misc_feature 9: note = /note="LNA nucleotide"
  misc_feature 13: note = /note="LNA nucleotide"
  misc_feature 15: note = /note="LNA nucleotide"
  misc_feature 2..5: note = /note="2'-O-methyl-nucleotide"
  misc_feature 6: note = /note="2'-O-methyl-nucleotide"
  misc_feature 8: note = /note="2'-O-methyl-nucleotide"
  misc_feature 10: note = /note="2'-O-methyl-nucleotide"
  misc_feature 11: note = /note="2'-O-methyl-nucleotide"
  misc_feature 12: note = /note="2'-O-methyl-nucleotide"
  misc_feature 14: note = /note="2'-O-methyl-nucleotide"
  source 1..15: mol_type = other RNA
ccctggcaatgtgat

SEQ ID NO: 93 - RNA, 15 nt, synthetic construct
  modified_base 1: mod_base = OTHER; note = thymine
  misc_feature 1..15: note = /note="combined DNA/RNA molecule" /note="Antagonist AntimiR-218"
  misc_feature 1..14: note = /note="Phosphorothioate bond"
  misc_feature 1: note = /note="LNA nucleotide"
  misc_feature 4: note = /note="LNA nucleotide"
  misc_feature 8: note = /note="LNA nucleotide"
  misc_feature 11: note = /note="LNA nucleotide"
  misc_feature 13: note = /note="LNA nucleotide"
  misc_feature 15: note = /note="LNA nucleotide"
  misc_feature 2..3: note = /note="2'-O-methyl-nucleotide"
  misc_feature 5..7: note = /note="2'-O-methyl-nucleotide"
  misc_feature 9..10: note = /note="2'-O-methyl-nucleotide"
  misc_feature 12: note = /note="2'-O-methyl-nucleotide"
  misc_feature 14: note = /note="2'-O-methyl-nucleotide"
  source 1..15: mol_type = other RNA
ttagatcaaggacaa

SEQ ID NO: 94 - RNA, 16 nt, synthetic construct
  modified_base 4: mod_base = OTHER; note = thymine
  modified_base 15: mod_base = OTHER; note = thymine
  misc_feature 1..16: note = /note="combined DNA/RNA molecule" /note="Antagonist AntimiR-SC"
  misc_feature 1..6: note = /note="LNA nucleotide"
  misc_feature 1..15: note = /note="Phosphorothioate bond"
  misc_feature 7..14: note = /note="2'-O-methyl-nucleotide"
  misc_feature 15..16: note = /note="LNA nucleotide"
  source 1..16: mol_type = other RNA
gcataatgactttatg

SEQ ID NO: 95 - RNA, 21 nt, synthetic construct
  modified_base 10: mod_base = OTHER; note = thymine
  misc_feature 1..21: note = FANA oligonucleotide AUM-miR-23b-l
  misc_feature 1..20: note = /note="Phosphorothioate bond"
  misc_feature 1: note = /note="2'-fluoroarabinonucleotide"
  misc_feature 21: note = /note="2'-fluoroarabinonucleotide"
  source 1..21: mol_type = other RNA
ggtaatccctggcaatgtgat

SEQ ID NO: 96 - RNA, 21 nt, synthetic construct
  modified_base 6: mod_base = OTHER; note = thymine
  modified_base 10: mod_base = OTHER; note = thymine
  modified_base 16: mod_base = OTHER; note = thymine
  modified_base 18: mod_base = OTHER; note = thymine
  misc_feature 1..21: note = FANA oligonucleotide AUM-miR-23b-2
  misc_feature 1..20: note = /note="Phosphorothioate bond"
  misc_feature 1: note = /note="2'-fluoroarabinonucleotide"
  misc_feature 21: note = /note="2'-fluoroarabinonucleotide"
  source 1..21: mol_type = other RNA
ggtaatccctggcaatgtgat

SEQ ID NO: 97 - RNA, 21 nt, synthetic construct
  misc_feature 1..21: note = FANA oligonucleotide AUM-miR-23b-3
  misc_feature 1..20: note = /note="Phosphorothioate bond"
  misc_feature 1: note = /note="2'-fluoroarabinonucleotide"
  misc_feature 21: note = /note="2'-fluoroarabinonucleotide"
  source 1..21: mol_type = other RNA
ggtaatccctggcaatgtgat

SEQ ID NO: 98 - RNA, 21 nt, synthetic construct
  modified_base 6: mod_base = OTHER; note = thymine
  modified_base 10: mod_base = OTHER; note = thymine
  modified_base 16: mod_base = OTHER; note = thymine
  modified_base 18: mod_base = OTHER; note = thymine
  misc_feature 1..21: note = FANA oligonucleotide AUM-miR-23b-4
  misc_feature 1..20: note = /note="Phosphorothioate bond"
  misc_feature 1: note = /note="2'-fluoroarabinonucleotide"
  misc_feature 21: note = /note="2'-fluoroarabinonucleotide"
  source 1..21: mol_type = other RNA
ggtaatccctggcaatgtgat

SEQ ID NO: 99 - RNA, 21 nt, synthetic construct
  modified_base 8: mod_base = OTHER; note = thymine
  modified_base 12: mod_base = OTHER; note = thymine
  misc_feature 1..21: note = FANA oligonucleotide AUM-miR-218-1
  misc_feature 1..20: note = /note="Phosphorothioate bond"
  misc_feature 1: note = /note="2'-fluoroarabinonucleotide"
  misc_feature 21: note = /note="2'-fluoroarabinonucleotide"
  source 1..21: mol_type = other RNA
acatggttagatcaagcacaa

SEQ ID NO: 100 - RNA, 21 nt, synthetic construct
  modified_base 4: mod_base = OTHER; note = thymine
  modified_base 12: mod_base = OTHER; note = thymine
  misc_feature 1..21: note = FANA oligonucleotide AUM-miR-218-2
  misc_feature 1..20: note = /note="Phosphorothioate bond"
  misc_feature 1: note = /note="2'-fluoroarabinonucleotide"
  misc_feature 21: note = /note="2'-fluoroarabinonucleotide"
  source 1..21: mol_type = other RNA
acatggttagatcaagcacaa

SEQ ID NO: 101 - RNA, 21 nt, synthetic construct
  misc_feature 1..21: note = FANA oligonucleotide AUM-miR-218-3
  misc_feature 1..20: note = /note="Phosphorothioate bond"
  misc_feature 1: note = /note="2'-fluoroarabinonucleotide"
  misc_feature 21: note = /note="2'-fluoroarabinonucleotide"
  source 1..21: mol_type = other RNA
acatggttagatcaagcacaa

SEQ ID NO: 102 - RNA, 21 nt, synthetic construct
  modified_base 4: mod_base = OTHER; note = thymine
  modified_base 8: mod_base = OTHER; note = thymine
  modified_base 12: mod_base = OTHER; note = thymine
  misc_feature 1..21: note = FANA oligonucleotide AUM-miR-218-4
  misc_feature 1..20: note = /note="Phosphorothioate bond"
  misc_feature 1: note = /note="2'-fluoroarabinonucleotide"
  misc_feature 21: note = /note="2'-fluoroarabinonucleotide"
  source 1..21: mol_type = other RNA
acatggttagatcaagcacaa

SEQ ID NO: 103 - RNA, 21 nt, synthetic construct
  modified_base 8: mod_base = OTHER; note = thymine
  modified_base 10: mod_base = OTHER; note = thymine
  modified_base 13: mod_base = OTHER; note = thymine
  misc_feature 1..21: note = FANA oligonucleotide AUM-SC-1
  misc_feature 1..20: note = /note="Phosphorothioate bond"
  misc_feature 1: note = /note="2'-fluoroarabinonucleotide"
  misc_feature 21: note = /note="2'-fluoroarabinonucleotide"
  source 1..21: mol_type = other RNA
atatccttgtcgtatcccagt

SEQ ID NO: 104 - RNA, 21 nt, synthetic construct
  misc_feature 1..21: note = FANA oligonucleotide AUM-SC-2
  misc_feature 1..20: note = /note="Phosphorothioate bond"
  misc_feature 1: note = /note="2'-fluoroarabinonucleotide"
  misc_feature 21: note = /note="2'-fluoroarabinonucleotide"
  source 1..21: mol_type = other RNA
  modified_base 8: mod_base = OTHER; note = thymine
  modified_base 10: mod_base = OTHER; note = thymine
  modified_base 13: mod_base = OTHER; note = thymine
atatccttgtcgtatcccagt